European Patent Application EP 4 282 876 A1, published November 29, 2023. Title: Uricase-Albumin conjugate and its manufacturing method, and use thereof. Applicant: Proabtech. The sequence listing filed with the application follows.

SEQUENCE LISTING (167 sequences)

SEQ ID NO: 1 - protein, 301 aa, Aspergillus Flavus
SAVKAARYGKDNVRVYKVHKDEKTGVQTVYEMTVCVLLEGEIETSYTKADNSVIVATDSIKNTIYITAKQNPVTPPELFGSILGTHFIEKYNHIHAAHVNIVCHRWTRMDIDGKPHPHSFIRDSEEKRNVQVDVVEGKGIDIKSSLSGLTVLKSTNSQFWGFLRDEYTTLKETWDRILSTDVDATWQWKNFSGLQEVRSHVPKFDATWATAREVTLKTFAEDNSASVQATMYKMAEQILARQQLIETVEYSLPNKHYFEIDLSWHKGLQNTGKNAEVFAPQSDPNGLIKCTVGRSSLKSKL

SEQ ID NO: 2 - protein, 301 aa, Artificial Sequence
  Asp.Uox Variant Subunit (G137)
  MISC_FEATURE (1)..(301): Xaa is unnatural amino acid containing tetrazine functional group, and/or triazine functional group.
SAVKAARYGKDNVRVYKVHKDEKTGVQTVYEMTVCVLLEGEIETSYTKADNSVIVATDSIKNTIYITAKQNPVTPPELFGSILGTHFIEKYNHIHAAHVNIVCHRWTRMDIDGKPHPHSFIRDSEEKRNVQVDVVEXKGIDIKSSLSGLTVLKSTNSQFWGFLRDEYTTLKETWDRILSTDVDATWQWKNFSGLQEVRSHVPKFDATWATAREVTLKTFAEDNSASVQATMYKMAEQILARQQLIETVEYSLPNKHYFEIDLSWHKGLQNTGKNAEVFAPQSDPNGLIKCTVGRSSLKSKL

SEQ ID NO: 3 - protein, 301 aa, Artificial Sequence
  Asp.Uox Variant Subunit
  MISC_FEATURE (1)..(301): Xaa is unnatural amino acid containing tetrazine functional group, and/or triazine functional group.
SAVKAARYGKDNVRVYKVHKDXKTGVQTVYEMTVCVLLEGEIETSYTKADNSVIVATDSIKNTIYITAKQNPVTPPELFGSILGTHFIEKYNHIHAAHVNIVCHRWTRMDIDGKPHPHSFIRDSEEKRNVQVDVVEGKGIDIKSSLSGLTVLKSTNSQFWGFLRDEYTTLKETWDRILSTDVDATWQWKNFSGLQEVRSHVPKFDATWATAREVTLKTFAEDNSASVQATMYKMAEQILARQQLIETVEYSLPNKHYFEIDLSWHKGLQNTGKNAEVFAPQSDPNGLIKCTVGRSSLKSKL

SEQ ID NO: 4 - protein, 301 aa, Artificial Sequence
  Asp.Uox Variant Subunit
  MISC_FEATURE (1)..(301): Xaa is unnatural amino acid containing tetrazine functional group, and/or triazine functional group.
SAVKAARYGKDNVRVYKVHKDEKTGVQTVYEMTVCVLLEGEIETSYTKADNSVIVATDSIKNTIYITAKQNPVTPPELFGSILGTHFIEKYXHIHAAHVNIVCHRWTRMDIDGKPHPHSFIRDSEEKRNVQVDVVEGKGIDIKSSLSGLTVLKSTNSQFWGFLRDEYTTLKETWDRILSTDVDATWQWKNFSGLQEVRSHVPKFDATWATAREVTLKTFAEDNSASVQATMYKMAEQILARQQLIETVEYSLPNKHYFEIDLSWHKGLQNTGKNAEVFAPQSDPNGLIKCTVGRSSLKSKL

SEQ ID NO: 5 - protein, 301 aa, Artificial Sequence
  Asp.Uox Variant Subunit
  MISC_FEATURE (1)..(301): Xaa is unnatural amino acid containing tetrazine functional group, and/or triazine functional group.
SAVKAARYGKDNVRVYKVHKDEXTGVQTVYEMTVCVLLEGEIETSYTKADNSVIVATDSIKNTIYITAKQNPVTPPELFGSILGTHFIEKYNHIHAAHVNIVCHRWTRMDIDGKPHPHSFIRDSEEKRNVQVDVVEGKGIDIKSSLSGLTVLKSTNSQFWGFLRDEYTTLKETWDRILSTDVDATWQWKNFSGLQEVRSHVPKFDATWATAREVTLKTFAEDNSASVQATMYKMAEQILARQQLIETVEYSLPNKHYFEIDLSWHKGLQNTGKNAEVFAPQSDPNGLIKCTVGRSSLKSKL

SEQ ID NO: 6 - protein, 301 aa, Artificial Sequence
  Asp.Uox Variant Subunit
  MISC_FEATURE (1)..(301): Xaa is unnatural amino acid containing tetrazine functional group, and/or triazine functional group.
SAVKAARYGKDNVRVYKVHKDEKTGVQTVYEMTVCVLLEGEIETSYTKADNSVIVATDSIKNTIYITAKQNPVTPPELFGSILGTHFIEKYNHIHAAHVNIVCHRWTRMDIDGKPHPHSFIRDSEEKRNVQVDVVEGKGIDIKSSLSGLTVLKSTNSQFWGFLRDEYTTLKETWDRILSTDVDATWQWKNFSGLQEVRSHVPKFDATWATAREVTLKTFAEDNSASVQATMYKMAEQILARQQLIETVEYSLPNKHYFEIDLSWHKGLQNTGKNAEVFAPQSDPNGLIKCTVGRXSLKSKL

SEQ ID NO: 7 - protein, 301 aa, Artificial Sequence
  Asp.Uox Variant Subunit
  MISC_FEATURE (1)..(301): Xaa is unnatural amino acid containing tetrazine functional group, and/or triazine functional group.
SAVKAARYGKDNVRVYKVHKDEKTGVQTVYEMTVCVLLEGEIETSYTKADNSVIVATDSIKNTIYITAKQNPVTPPELFGSILGTHFIEKYNHIHAAHVNIVCHRWTRMDIDXKPHPHSFIRDSEEKRNVQVDVVEGKGIDIKSSLSGLTVLKSTNSQFWGFLRDEYTTLKETWDRILSTDVDATWQWKNFSGLQEVRSHVPKFDATWATAREVTLKTFAEDNSASVQATMYKMAEQILARQQLIETVEYSLPNKHYFEIDLSWHKGLQNTGKNAEVFAPQSDPNGLIKCTVGRSSLKSKL

SEQ ID NO: 8 - protein, 301 aa, Artificial Sequence
  Asp.Uox Variant Subunit
  MISC_FEATURE (1)..(301): Xaa is unnatural amino acid containing tetrazine functional group, and/or triazine functional group.
SAVKAARYGKDNVRVYKVHKDEKTGVQTVYEMTVCVLLEGEIETSYTKADNSVIVATDSIKNTIYITAKQNPVTPPELFGSILGTHFIEKYNHIHAAHVNIVCHRWTRMDIDGKPHPHSFIRDSEEKRNVQVDVVEGKGIDIKSSLSGLTVLKSTNSQFWGFLRDEYTTLKETWDRILSTDVDATWQWKNFSGLQEVRSHVPKFDATWATAREVTLKTFAEDNSASVQATMYKMAEQILARQQLIETVEYSLPNKHYFEIDLSWHKGLQNTGXNAEVFAPQSDPNGLIKCTVGRSSLKSKL

SEQ ID NO: 9 - protein, 301 aa, Artificial Sequence
  Asp.Uox Variant Subunit
  MISC_FEATURE (1)..(301): Xaa is unnatural amino acid containing tetrazine functional group, and/or triazine functional group.
SAVKAARYGKDNVRVYKVHKDEKTGVQTVYEMTVCVLLEGEIETSYTKADNSVIVATDSIKNTIYITAKQNPVTPPELFGSILGTHFIEKYNHIHAAHVNIVCHRWTRMDIDGKPHPHSFIRDSEEKRNVQVDVVEGKGIDIKSSLSGLTVLKSTNSQFWGFLRDEYTTLXETWDRILSTDVDATWQWKNFSGLQEVRSHVPKFDATWATAREVTLKTFAEDNSASVQATMYKMAEQILARQQLIETVEYSLPNKHYFEIDLSWHKGLQNTGKNAEVFAPQSDPNGLIKCTVGRSSLKSKL

SEQ ID NO: 10 - protein, 301 aa, Artificial Sequence
  Asp.Uox Variant Subunit
  MISC_FEATURE (1)..(301): Xaa is unnatural amino acid containing tetrazine functional group, and/or triazine functional group.
SAVKAARYGKDNVRVYKVHKDEKTGVQTVYEMTVCVLLEGEIETSYTKADNSVIVATDSIKNTIYITAKQNPVTPPELFGSILGTHFIEKYNHIHAAHVNIVCHRWTRMDIDGKPHPHSFIRDSEEKRNVQVDVVEGKGIDIKSSLSGLTVLKSTNSQFWGFLRDEYTTLKETWDRILSTDVDATWQWKNFSGLQEVRSHVPKFDATWATAREVTLKTFAEDNSASVQATMYKMAEQILXRQQLIETVEYSLPNKHYFEIDLSWHKGLQNTGKNAEVFAPQSDPNGLIKCTVGRSSLKSKL

SEQ ID NO: 11 - protein, 301 aa, Artificial Sequence
  Asp.Uox Variant Subunit
  MISC_FEATURE (1)..(301): Xaa is unnatural amino acid containing tetrazine functional group, and/or triazine functional group.
SAVKAARYGKDNVRVYKVHKDEKTGVQTVYEMTVCVLLEGEIETSYTKADNSVIVATDSIKNTIYITAKQNPVTPPELFGSILGTHFIXKYNHIHAAHVNIVCHRWTRMDIDGKPHPHSFIRDSEEKRNVQVDVVEGKGIDIKSSLSGLTVLKSTNSQFWGFLRDEYTTLKETWDRILSTDVDATWQWKNFSGLQEVRSHVPKFDATWATAREVTLKTFAEDNSASVQATMYKMAEQILARQQLIETVEYSLPNKHYFEIDLSWHKGLQNTGKNAEVFAPQSDPNGLIKCTVGRSSLKSKL

SEQ ID NO: 12 - protein, 301 aa, Artificial Sequence
  Asp.Uox Variant Subunit
  MISC_FEATURE (1)..(301): Xaa is unnatural amino acid containing tetrazine functional group, and/or triazine functional group.
SAVKAARYGKDNVRVYKVHKDEKTGVQTVYEMTVCVLLEGEIETSYTKADNSVIVATDSIKNTIYITAKQNPVTPPELFGSILGTHFIEKYNHIHAAHVNIVCHRWTRMDIDGKPHPHSFIRDSEEKRNVQVDVVEGKGIDIKSSLSGLTVLKSTNSQFWGFLRDEYTTLKETWDRILSTDVDATWQWKNFSGLQEVRSHVPKFDATWATAREVTLKTFAEDNSASVQATMYKMAEQILARQQLIETVEYSLPNKHYFEIDLSWHXGLQNTGKNAEVFAPQSDPNGLIKCTVGRSSLKSKL

SEQ ID NO: 13 - protein, 301 aa, Artificial Sequence
  Asp.Uox Variant Subunit
  MISC_FEATURE (1)..(301): Xaa is unnatural amino acid containing tetrazine functional group, and/or triazine functional group.
SAVKAARYGKDNVRVYKVHKDEKXGVQTVYEMTVCVLLEGEIETSYTKADNSVIVATDSIKNTIYITAKQNPVTPPELFGSILGTHFIEKYNHIHAAHVNIVCHRWTRMDIDGKPHPHSFIRDSEEKRNVQVDVVEGKGIDIKSSLSGLTVLKSTNSQFWGFLRDEYTTLKETWDRILSTDVDATWQWKNFSGLQEVRSHVPKFDATWATAREVTLKTFAEDNSASVQATMYKMAEQILARQQLIETVEYSLPNKHYFEIDLSWHKGLQNTGKNAEVFAPQSDPNGLIKCTVGRSSLKSKL

SEQ ID NO: 14 - protein, 301 aa, Artificial Sequence
  Asp.Uox Variant Subunit
  MISC_FEATURE (1)..(301): Xaa is unnatural amino acid containing tetrazine functional group, and/or triazine functional group.
SAVKAARYGKDNVRVYKVHKDEKTGVQTVYEMTVCVLLEGEIETSYTXADNSVIVATDSIKNTIYITAKQNPVTPPELFGSILGTHFIEKYNHIHAAHVNIVCHRWTRMDIDGKPHPHSFIRDSEEKRNVQVDVVEGKGIDIKSSLSGLTVLKSTNSQFWGFLRDEYTTLKETWDRILSTDVDATWQWKNFSGLQEVRSHVPKFDATWATAREVTLKTFAEDNSASVQATMYKMAEQILARQQLIETVEYSLPNKHYFEIDLSWHKGLQNTGKNAEVFAPQSDPNGLIKCTVGRSSLKSKL

SEQ ID NO: 15 - protein, 301 aa, Artificial Sequence
  Asp.Uox Variant Subunit
  MISC_FEATURE (1)..(301): Xaa is unnatural amino acid containing tetrazine functional group, and/or triazine functional group.
SAVKAARYGKDNVRVYKVHKDEKTGVQTVYEMTVCVLLEGEIETSYTKADNSVIVATDSIKNTIYITAKQNPVTPPELFGSILGTHFIEKYNHIHAAHVNIVCHRWTRMDIDGKPHPHSFIRDSEEKRNVQVDVVEGKGIDIKSSLSGLTVLKSTNSQFWGFLRDEYTTLKETWDRILSTDVDATWQWKNFXGLQEVRSHVPKFDATWATAREVTLKTFAEDNSASVQATMYKMAEQILARQQLIETVEYSLPNKHYFEIDLSWHKGLQNTGKNAEVFAPQSDPNGLIKCTVGRSSLKSKL

SEQ ID NO: 16 - protein, 301 aa, Artificial Sequence
  Asp.Uox Variant Subunit
SAVKAARYGKDNVRVYKVHKDEKTGVQTVYEMTVCVLLEGEIETSYTKADNSVIVATDSIKNTIYITAKQNPVTPPELFGSILGTHFIEKYNHIHAAHVNIVCHRWTRMDIDGKPHPHSFIRDSEEKRNVQVDVVEGKGIDIKSSLSGLTVLKSTNSQFWGFLRDEYTTLKETWDRILSTDVDATWQWKNFSGLQEVRSHVXKFDATWATAREVTLKTFAEDNSASVQATMYKMAEQILARQQLIETVEYSLPNKHYFEIDLSWHKGLQNTGKNAEVFAPQSDPNGLIKCTVGRSSLKSKL

SEQ ID NO: 17 - protein, 301 aa, Artificial Sequence
  Asp.Uox Variant Subunit
SAVKAARYGKDNVRVYKVHKDEKTGVQTVYEMTVCVLLEGEIETSYTKADNSVIVATDSIKNTIYITAKQNPVTPPELFGSILGTHFIEKYNHIHAAHVNIVCHRWTRMXIDGKPHPHSFIRDSEEKRNVQVDVVEGKGIDIKSSLSGLTVLKSTNSQFWGFLRDEYTTLKETWDRILSTDVDATWQWKNFSGLQEVRSHVPKFDATWATAREVTLKTFAEDNSASVQATMYKMAEQILARQQLIETVEYSLPNKHYFEIDLSWHKGLQNTGKNAEVFAPQSDPNGLIKCTVGRSSLKSKL

SEQ ID NO: 18 - protein, 301 aa, Artificial Sequence
  Asp.Uox Variant Subunit
  MISC_FEATURE (1)..(301): Xaa is unnatural amino acid containing tetrazine functional group, and/or triazine functional group.
SAVKAARYGKDNVRVYKVHKDEKTGVQTVYEMTVCVLLEGEIETSYTKADNSVIVATDSIKNTIYITAKQNPVTPPELFGSILGTHFIEKYNHIHAAHVNIVCHRWTRMDIDGKPHPHSFIRDSEEKRNVQVDVVEGKGIDIKSSLSGLTVLKSTNSQFWGFLRDEYTTLKETWDRILSTDVDATWQWKNFSGLQEVRSHVPKFDATWATAREVTLKTFAEDNSASVQATMYKMAEQILARQXLIETVEYSLPNKHYFEIDLSWHKGLQNTGKNAEVFAPQSDPNGLIKCTVGRSSLKSKL

SEQ ID NO: 19 - protein, 301 aa, Artificial Sequence
  Asp.Uox Variant Subunit
SAVKAARYGKDNVRVYKVHKDEKTGVQTVYEMTVCVLLEGEIETSYTKADNSVIVATDSIKNTIYITAKQNPVTPPELFGSILGTHFIEKYNHIHAAHVNIVCHRWTRMDIDGKPHPHSFIRDSEEKRNVQVDVVEGKGIDIKSSLSGLTVLKSTNSQFWGFLRDEYTTLKETWDRILSTDVDATWQWKNFSGLXEVRSHVPKFDATWATAREVTLKTFAEDNSASVQATMYKMAEQILARQQLIETVEYSLPNKHYFEIDLSWHKGLQNTGKNAEVFAPQSDPNGLIKCTVGRSSLKSKL

SEQ ID NO: 20 - protein, 301 aa, Artificial Sequence
  Asp.Uox Variant Subunit
SAVKAARYGKDNVRVYKVHKDEKTGVQTVYEMTVCVLLEGEIETSYTKADNSVIVATDSIKNTIYITAKQNPVTPPELFGSILGTHFIEKYNHIHAAHVNIVCHRWTRMDIDGKPHPHSFIRDSEEKRNVQVDVVEGXGIDIKSSLSGLTVLKSTNSQFWGFLRDEYTTLKETWDRILSTDVDATWQWKNFSGLQEVRSHVPKFDATWATAREVTLKTFAEDNSASVQATMYKMAEQILARQQLIETVEYSLPNKHYFEIDLSWHKGLQNTGKNAEVFAPQSDPNGLIKCTVGRSSLKSKL

SEQ ID NO: 21 - protein, 301 aa, Artificial Sequence
  Asp.Uox Variant Subunit
  MISC_FEATURE (1)..(301): Xaa is unnatural amino acid containing tetrazine functional group, and/or triazine functional group.
SAVKAARYGKDNVRVYKVHKDEKTGVQTVYEMTVCVLLEGEIETSYTKADNSVIVATDSIKNTIYITAKQNPVTPPELFGSILGTHFIEKYNHIHAAHVNIVCHRWTRMDIDGKXHPHSFIRDSEEKRNVQVDVVEGKGIDIKSSLSGLTVLKSTNSQFWGFLRDEYTTLKETWDRILSTDVDATWQWKNFSGLQEVRSHVPKFDATWATAREVTLKTFAEDNSASVQATMYKMAEQILARQQLIETVEYSLPNKHYFEIDLSWHKGLQNTGKNAEVFAPQSDPNGLIKCTVGRSSLKSKL

SEQ ID NO: 22 - protein, 301 aa, Artificial Sequence
  Asp.Uox Variant Subunit
SAVKAARYGKDNVRVYKVHKDEKTGVQTVYEMTVCVLLEGEIETSYTKADNSVIVATDSIKNTIYITAKQNPVTPPELFGSILGTHFIEKYNHIHAAHVNIVCHRWTRMDIDGKPHPHSFIRDSEEKRNVQVDVVEGKGIDIKSSLSGLTVLKSTNSQFWGFLRDEYTTLKETWDRILSTDVDATWQWKNFSGLQEVRXHVPKFDATWATAREVTLKTFAEDNSASVQATMYKMAEQILARQQLIETVEYSLPNKHYFEIDLSWHKGLQNTGKNAEVFAPQSDPNGLIKCTVGRSSLKSKL

SEQ ID NO: 23 - protein, 301 aa, Artificial Sequence
  Asp.Uox Variant Subunit
SAVKAARYGKDNVRVYKVHKDEKTGVQTVYEMTVCVLLEGEIETSYTKADNSVIVATDSIKNTIYITAKQNPVTPPELFGSILGTHFIEKYNHIHAAHVNIVCHRWTRMDIDGKPHPHSFIRDSEEKRNVQVDVVEGKGIDIKSSLSGLTVLKSTNSQFWGFLRDEYTTLKETWDRILSTDVDATWQWKNFSGLQEVRSHVPKFDATWATAREVTLKTFAEDNSASVQATMYKMAEQILARQQLIETVEYSLPNKHYFEIDLSWHKGLQNTXKNAEVFAPQSDPNGLIKCTVGRSSLKSKL

SEQ ID NO: 24 - protein, 301 aa, Artificial Sequence
  Asp.Uox Variant Subunit
  MISC_FEATURE (1)..(301): Xaa is unnatural amino acid containing tetrazine functional group, and/or triazine functional group.
SAVXAARYGKDNVRVYKVHKDEKTGVQTVYEMTVCVLLEGEIETSYTKADNSVIVATDSIKNTIYITAKQNPVTPPELFGSILGTHFIEKYNHIHAAHVNIVCHRWTRMDIDGKPHPHSFIRDSEEKRNVQVDVVEGKGIDIKSSLSGLTVLKSTNSQFWGFLRDEYTTLKETWDRILSTDVDATWQWKNFSGLQEVRSHVPKFDATWATAREVTLKTFAEDNSASVQATMYKMAEQILARQQLIETVEYSLPNKHYFEIDLSWHKGLQNTGKNAEVFAPQSDPNGLIKCTVGRSSLKSKL

SEQ ID NO: 25 - protein, 301 aa, Artificial Sequence
  Asp.Uox Variant Subunit
SAVKAARYGKDNVRVYKVHKDEKTGVQTVYEMTVCVLLEGEIETSYTKADNSVIVATDSIKNTIYITAKQNPVTPPELFGSILGTHFIEKYNHIHAAHVNIVCHRWTRMDIXGKPHPHSFIRDSEEKRNVQVDVVEGKGIDIKSSLSGLTVLKSTNSQFWGFLRDEYTTLKETWDRILSTDVDATWQWKNFSGLQEVRSHVPKFDATWATAREVTLKTFAEDNSASVQATMYKMAEQILARQQLIETVEYSLPNKHYFEIDLSWHKGLQNTGKNAEVFAPQSDPNGLIKCTVGRSSLKSKL

SEQ ID NO: 26 - protein, 301 aa, Artificial Sequence
  Asp.Uox Variant Subunit
SAVKAARYGKDNVRVYKVHKDEKTGVQTVYEMTVCVLLEGEIETSYTKADNSVIVATDSIKNTIYITAKQNPVTPPELFGSILGTHFIEKYNHIHAAHVNIVCHRWTRMDIDGKPHPHSFIRDSEEKRNVQVDVVEGKGIDIKSSLSGLTVLKSTNSQFWGFLRDEYTTLKETWDRILSTDVDATWQWKNFSGLQEVRSHVPKFDATWATAREVTLKTFAEDNSASVQATMYKMAEQILARQQLIETVEYSLPNKHYFEIDLSWHKXLQNTGKNAEVFAPQSDPNGLIKCTVGRSSLKSKL

SEQ ID NO: 27 - protein, 301 aa, Artificial Sequence
  Asp.Uox Variant Subunit
  MISC_FEATURE (1)..(301): Xaa is unnatural amino acid containing tetrazine functional group, and/or triazine functional group.
SAVKAARYGKDNVRVYKVHKDEKTGVQTVYEMTVCVLLEGEIETSYTKADNSVIVATDSIKNTIYITAKQNPVTPPELFGSILGTHFIEKYNHIHAAHVNIVCHRWTRMDIDGXPHPHSFIRDSEEKRNVQVDVVEGKGIDIKSSLSGLTVLKSTNSQFWGFLRDEYTTLKETWDRILSTDVDATWQWKNFSGLQEVRSHVPKFDATWATAREVTLKTFAEDNSASVQATMYKMAEQILARQQLIETVEYSLPNKHYFEIDLSWHKGLQNTGKNAEVFAPQSDPNGLIKCTVGRSSLKSKL

SEQ ID NO: 28 - protein, 301 aa, Artificial Sequence
  Asp.Uox Variant Subunit
SAVKAARYGKDNVRVYKVHKDEKTGVQTVYEMTVCVLLEGEIETSYTKADNSVIVATDSIKNTIYITAKXNPVTPPELFGSILGTHFIEKYNHIHAAHVNIVCHRWTRMDIDGKPHPHSFIRDSEEKRNVQVDVVEGKGIDIKSSLSGLTVLKSTNSQFWGFLRDEYTTLKETWDRILSTDVDATWQWKNFSGLQEVRSHVPKFDATWATAREVTLKTFAEDNSASVQATMYKMAEQILARQQLIETVEYSLPNKHYFEIDLSWHKGLQNTGKNAEVFAPQSDPNGLIKCTVGRSSLKSKL

SEQ ID NO: 29 - protein, 301 aa, Artificial Sequence
  Asp.Uox Variant Subunit
SAVKAARYGKDNVRVYKVHKDEKTGVQTVYEMTVCVLLEGEIETSYTKADNSVIVATDSIKNTIYITAKQNPVTPPELFGSILGTHFIEKYNHIHAAHVNIVCHRWTRMDIDGKPHPHSFIRDSEEKRNVQVDVVEGKGIDIKSSLSGLTVLKSTNSQFWGFLRDEYTTLKETXDRILSTDVDATWQWKNFSGLQEVRSHVPKFDATWATAREVTLKTFAEDNSASVQATMYKMAEQILARQQLIETVEYSLPNKHYFEIDLSWHKGLQNTGKNAEVFAPQSDPNGLIKCTVGRSSLKSKL

SEQ ID NO: 30 - protein, 301 aa, Artificial Sequence
  Asp.Uox Variant Subunit
  MISC_FEATURE (1)..(301): Xaa is unnatural amino acid containing tetrazine functional group, and/or triazine functional group.
SAVKAARYGKDNVRVYKVHKDEKTGVQTVYEMTVCVLLEGEIETSYTKADNSVIVATDSIKNTIYITAKQNPVTPPELFGSILGTHFIEKYNHIHAAHVNIVCHRWTRMDIDGKPHPHSFIRDSEEKRNVQVDVVEGKGIDIKSSLSGLTVLKSTNSQFWGFLRDEYTTLKETWDRILSTDVDATWQWKNFSGLQEVRSHVPKFDATWATAREVTLKTFAEDXSASVQATMYKMAEQILARQQLIETVEYSLPNKHYFEIDLSWHKGLQNTGKNAEVFAPQSDPNGLIKCTVGRSSLKSKL

SEQ ID NO: 31 - protein, 301 aa, Artificial Sequence
  Asp.Uox Variant Subunit
SAVKAARYGKDNVRVYKVHKDEKTGVQTVYEMTVCVLLEGXIETSYTKADNSVIVATDSIKNTIYITAKQNPVTPPELFGSILGTHFIEKYNHIHAAHVNIVCHRWTRMDIDGKPHPHSFIRDSEEKRNVQVDVVEGKGIDIKSSLSGLTVLKSTNSQFWGFLRDEYTTLKETWDRILSTDVDATWQWKNFSGLQEVRSHVPKFDATWATAREVTLKTFAEDNSASVQATMYKMAEQILARQQLIETVEYSLPNKHYFEIDLSWHKGLQNTGKNAEVFAPQSDPNGLIKCTVGRSSLKSKL

SEQ ID NO: 32 - protein, 301 aa, Artificial Sequence
  Asp.Uox Variant Subunit
SAVKAARYGKDNVRVYKVHKDEKTGVQTVYEMTVCVLLEGEIETSYTKADNSVIVATDSIKNTIYITAKQNPVTPPELFGSILGTHFIEKYNHIHAAHVNIVCHRWTRMDIDGKPHPHSFIRDSEEKRNVQVDVVEGKGIDIKSSLSGLTVLKSTNSQFWGFLRDEYTTLKETWDRILSTDVDATWQWKNFSGLQEVRSHVPKFDATWATAREVTLKTFAEDNSASVQATMYKMAEQILARQQLIETVEYSLPNKHYFEIXLSWHKGLQNTGKNAEVFAPQSDPNGLIKCTVGRSSLKSKL

SEQ ID NO: 33 - protein, 301 aa, Artificial Sequence
  Asp.Uox Variant Subunit
  MISC_FEATURE (1)..(301): Xaa is unnatural amino acid containing tetrazine functional group, and/or triazine functional group.
SAVKAARYGKDNVRVYKVHKDEKTXVQTVYEMTVCVLLEGEIETSYTKADNSVIVATDSIKNTIYITAKQNPVTPPELFGSILGTHFIEKYNHIHAAHVNIVCHRWTRMDIDGKPHPHSFIRDSEEKRNVQVDVVEGKGIDIKSSLSGLTVLKSTNSQFWGFLRDEYTTLKETWDRILSTDVDATWQWKNFSGLQEVRSHVPKFDATWATAREVTLKTFAEDNSASVQATMYKMAEQILARQQLIETVEYSLPNKHYFEIDLSWHKGLQNTGKNAEVFAPQSDPNGLIKCTVGRSSLKSKL

SEQ ID NO: 34 - protein, 301 aa, Artificial Sequence
  Asp.Uox Variant Subunit
SAVKAARYGKDNVRVYKVHKDEKTGVQTVYEMTVCVLLEGEIETSYTKADNXVIVATDSIKNTIYITAKQNPVTPPELFGSILGTHFIEKYNHIHAAHVNIVCHRWTRMDIDGKPHPHSFIRDSEEKRNVQVDVVEGKGIDIKSSLSGLTVLKSTNSQFWGFLRDEYTTLKETWDRILSTDVDATWQWKNFSGLQEVRSHVPKFDATWATAREVTLKTFAEDNSASVQATMYKMAEQILARQQLIETVEYSLPNKHYFEIDLSWHKGLQNTGKNAEVFAPQSDPNGLIKCTVGRSSLKSKL

SEQ ID NO: 35 - protein, 301 aa, Artificial Sequence
  Asp.Uox Variant Subunit
SAVKAARYGKDNVRVYKVHKDEKTGVQTVYEMTVCVLLEGEIETSYTKADNSVIVATDSIKNTIYITAKQNPVTPPELFGSILGTHFIEKYNHIHAAHVNIVCHRWTRMDIDGKPHPHSFIRDSEEKRNVQVDVVEGKGIDIKSSLSGLTVLKSTNSQFWGFLRDEYTTLKETWDRILSTDVDATWQWKNFSGLQEVRSHVPKFDATWATAREVTLKTFAEDNSASVQATMYKMAEQILAXQQLIETVEYSLPNKHYFEIDLSWHKGLQNTGKNAEVFAPQSDPNGLIKCTVGRSSLKSKL

SEQ ID NO: 36 - protein, 301 aa, Artificial Sequence
  Asp.Uox Variant Subunit
  MISC_FEATURE (1)..(301): Xaa is unnatural amino acid containing tetrazine functional group, and/or triazine functional group.
SAVKAARYGKDNVRVYKVHKDEKTGVQTVYEMTVCVLLEGEIETSYTKADNSVIVATDSIKNTIYITAKQNPVTPPELFGSILGTHFIEKYNHIHAAHVNIVCHRWTRMDIDGKPHPHSFIRDSEEKRNVQVDVVEGKGIDIKSSLSGLTVLKSTNSQFWGFLRDEYTTLKETWDRILSTDVDATWQWKNFSGLQEVRSHVPKFDATWATARXVTLKTFAEDNSASVQATMYKMAEQILARQQLIETVEYSLPNKHYFEIDLSWHKGLQNTGKNAEVFAPQSDPNGLIKCTVGRSSLKSKL

SEQ ID NO: 37 - protein, 301 aa, Artificial Sequence
  Asp.Uox Variant Subunit
SAVKAARYGKDNVRVYKVHKDEKTGVQTVYEMTVCVLLEGEIETSYTKADNSVIVATDSIKNTIYITAKQNPVTPPELFGSILGTHFIEKYNHIHAAHVNIVCHRWTRMDIDGKPHPHSFIRDSEEKRNVQVDVVEGKGIDIKSSLSGLTVLKSTNSQFWGFLRDEYTTLKETWDRILSTDVDATWQWKNFSGLQEVRSHVPKFDATWATAREVTLKTFAEDNSASVQATMYKMAEQILARQQLIETVEYSLPNKHYFEIDLSWHKGLQNTGKXAEVFAPQSDPNGLIKCTVGRSSLKSKL

SEQ ID NO: 38 - protein, 301 aa, Artificial Sequence
  Asp.Uox Variant Subunit
SAVKAARYGKDNVRVYKVHKDEKTGVQTVYEMTVCVLLEGEIETSYTKADNSVIVATDSIKNTIYITAKQNPVTPPELFGSILGTHFIEKYNHIHAAHVNIVCHRWTRMDIDGKPHPHSFIRDSEEKRNVQVDVVEGKGIDIKSSLSGLTVLKSTNSQFWGFLRDEYTTLKETWDRILSTDVDATWQWKNFSGLQEVRSHVPKFDATWATAREVTLKTFAXDNSASVQATMYKMAEQILARQQLIETVEYSLPNKHYFEIDLSWHKGLQNTGKNAEVFAPQSDPNGLIKCTVGRSSLKSKL

SEQ ID NO: 39 - protein, 301 aa, Artificial Sequence
  Asp.Uox Variant Subunit
  MISC_FEATURE (1)..(301): Xaa is unnatural amino acid containing tetrazine functional group, and/or triazine functional group.
SAVKAARYGKDNVRVYKVHKDEKTGVQTVYEMTVCVLLEGEIETSYTKADNSVIVATDSIKNTIYITAKQNPVTPPELFGSILGTHFIEKYNHIHAAHVNIVCHRWTRMDIDGKPHPHSFIRDSEEKRNVQVDVVEGKGIDIKSSLSGLTVLKSTNSQFWGFLRDEYTTLKETWDRILSTDVDATWQWKNFSGLQEVRSHVPKFDXTWATAREVTLKTFAEDNSASVQATMYKMAEQILARQQLIETVEYSLPNKHYFEIDLSWHKGLQNTGKNAEVFAPQSDPNGLIKCTVGRSSLKSKL

SEQ ID NO: 40 - protein, 301 aa, Artificial Sequence
  Asp.Uox Variant Subunit
SAVKAARYGKDNVRVYKVHKDEKTGVQTVYEMTVCVLLEGEIETSYTKADNSVIVATDSIKNTIYITAKQNPVTPPELFGSILGTHFIEKYNHIHAAHVNIVCHRWTRMDIDGKPHPHSFIRDSEEKRNVQVDVVEGKGIDIKSSLSGLTVLKSTNSQFWGFLRDEYTTLKETWDRILSTDVDATWQWKNFSGLQEVRSHVPKFDATWATAREVTLKTFAEDNSASVQATMYKMAXQILARQQLIETVEYSLPNKHYFEIDLSWHKGLQNTGKNAEVFAPQSDPNGLIKCTVGRSSLKSKL

SEQ ID NO: 41 - protein, 301 aa, Artificial Sequence
  Asp.Uox Variant Subunit
SAVKAARYGKDNVRVYKVHKDEKTGVQTVYEMTVCVLLEGEIETSYTKADNSVIVATDSIKNTIYITAKQNPVTPPELFGSILGTHFIEKYNHIHAAHVNIVCHRWTRMDIDGKPHPHSFIRDSEEKRNVQVDVVEGKGIDIKSSLSGLTVLKSTNSQFWGFLXDEYTTLKETWDRILSTDVDATWQWKNFSGLQEVRSHVPKFDATWATAREVTLKTFAEDNSASVQATMYKMAEQILARQQLIETVEYSLPNKHYFEIDLSWHKGLQNTGKNAEVFAPQSDPNGLIKCTVGRSSLKSKL

SEQ ID NO: 42 - protein, 301 aa, Artificial Sequence
  Asp.Uox Variant Subunit
  MISC_FEATURE (1)..(301): Xaa is unnatural amino acid containing tetrazine functional group, and/or triazine functional group.
SAVKAARYGKDNVRVYKVHKDEKTGVQTVYEMTVCVLLEGEIETSYTKADNSVIVATDSIKNTIYITAKQNPVTPPELFGSILGTHFIEKYNHIHAAHVNIVCHRWTRMDIDGKPHPHSFIRDSEEKRNVQVDVVEGKGIDIKSSLSGLTVLKSTNSQFWGFLRDEYTTLKETWDRILSTDVDATWQWKNFSGLQEVRSHVPKFDATWATAREVTLKTFAEDNSASVQATMYKMAEQILARQQLIETVEYSLPNKHYFEIDLSWHKGLXNTGKNAEVFAPQSDPNGLIKCTVGRSSLKSKL

SEQ ID NO: 43 - protein, 301 aa, Artificial Sequence
  Asp.Uox Variant Subunit
SAVKAARYGKDNVRVYKVHKDEKTGVQTVYEMTVCVLLEGEIETSYTKADNSVIVATDSIKNTIYITAKQNPVTPPELFGSILGTHFIEKYNHIHAAHVNIVCHRWTRMDIDGKPHPHSFIRDSEEKRNVQVDVVXGKGIDIKSSLSGLTVLKSTNSQFWGFLRDEYTTLKETWDRILSTDVDATWQWKNFSGLQEVRSHVPKFDATWATAREVTLKTFAEDNSASVQATMYKMAEQILARQQLIETVEYSLPNKHYFEIDLSWHKGLQNTGKNAEVFAPQSDPNGLIKCTVGRSSLKSKL

SEQ ID NO: 44 - protein, 301 aa, Artificial Sequence
  Asp.Uox Variant Subunit
SAVKAARYGKDNVRVYKVHKDEKTGVQTVYEMTVCVLLEGEIETSYTKADNSVIVATDSIKNTIYITAKQNPVTPPELFGSILGTHFIEKYNHIHAAHVNIVCHRWTRMDIDGKPHPHSFIRDSEEKRNVQVDVVEGKGIDIKSSLSGLTVLKSTNSQFWGFLRDEYTTLKETWDRILSTDVDATWQWKNFSGLQEVRSHVPKFDATWATAREVTLKTFAEDNSASVQATMYKMAEQILARQQLIETVEYSLPNKHYFXIDLSWHKGLQNTGKNAEVFAPQSDPNGLIKCTVGRSSLKSKL

SEQ ID NO: 45 - protein, 301 aa, Artificial Sequence
  Asp.Uox Variant Subunit
  MISC_FEATURE (1)..(301): Xaa is unnatural amino acid containing tetrazine functional group, and/or triazine functional group.
SAVKAARYGKDNVRVYKVHKDEKTGVQTVYEMTVCVLLEGEIETSYTKADNSVIVATDSIKNTIYITAKQNPVTPPELFGSILGTHFIEKYNHIHAAHVNIVCHRWTRMDIDGKPHPHSFIRDSEEKRNVQVDVVEGKGIDIKSSLSGLTVLKSTNSQFWGFLRDEYTTLKETWDRILSTDVDATWQWKNFSGLQEVRSHVPKFDATWATAREVTLKTFAEDNSASVQATMYKMAEQILARQQLIXTVEYSLPNKHYFEIDLSWHKGLQNTGKNAEVFAPQSDPNGLIKCTVGRSSLKSKL

SEQ ID NO: 46 - protein, 301 aa, Artificial Sequence
  Asp.Uox Variant Subunit
SAVKAARYGKDNVRVYKVHKDEKTGVQTVYEMTVCVLLEGEIETSYTKXDNSVIVATDSIKNTIYITAKQNPVTPPELFGSILGTHFIEKYNHIHAAHVNIVCHRWTRMDIDGKPHPHSFIRDSEEKRNVQVDVVEGKGIDIKSSLSGLTVLKSTNSQFWGFLRDEYTTLKETWDRILSTDVDATWQWKNFSGLQEVRSHVPKFDATWATAREVTLKTFAEDNSASVQATMYKMAEQILARQQLIETVEYSLPNKHYFEIDLSWHKGLQNTGKNAEVFAPQSDPNGLIKCTVGRSSLKSKL

SEQ ID NO: 47 - protein, 301 aa, Artificial Sequence
  Asp.Uox Variant Subunit
SAVKAARYGKDNVRVYKVHKDEKTGVQTVYEMTVCVLLEGEIETSYTKADNSVIVATDSIKNTIYITAKQNPVTPPELFGSILGTHFIEKYNHIHAAHVNIVCHRWTRMDIDGKPHPHSFIRDSEEKRNVQVDVVEGKGIDIKSSLSXLTVLKSTNSQFWGFLRDEYTTLKETWDRILSTDVDATWQWKNFSGLQEVRSHVPKFDATWATAREVTLKTFAEDNSASVQATMYKMAEQILARQQLIETVEYSLPNKHYFEIDLSWHKGLQNTGKNAEVFAPQSDPNGLIKCTVGRSSLKSKL

SEQ ID NO: 48 - protein, 301 aa, Artificial Sequence
  Asp.Uox Variant Subunit
  MISC_FEATURE (1)..(301): Xaa is unnatural amino acid containing tetrazine functional group, and/or triazine functional group.
SAVKAARYGKDNVRVYKVXKDEKTGVQTVYEMTVCVLLEGEIETSYTKADNSVIVATDSIKNTIYITAKQNPVTPPELFGSILGTHFIEKYNHIHAAHVNIVCHRWTRMDIDGKPHPHSFIRDSEEKRNVQVDVVEGKGIDIKSSLSGLTVLKSTNSQFWGFLRDEYTTLKETWDRILSTDVDATWQWKNFSGLQEVRSHVPKFDATWATAREVTLKTFAEDNSASVQATMYKMAEQILARQQLIETVEYSLPNKHYFEIDLSWHKGLQNTGKNAEVFAPQSDPNGLIKCTVGRSSLKSKL

SEQ ID NO: 49 - protein, 301 aa, Artificial Sequence
  Asp.Uox Variant Subunit
SAVKAARYGKDNVRVYKVHKDEKTGVQTVYEMTVCVLLEGEIETSYTKADNSVIVATDSIKNTIYITAKQNPVTPPELFGSILGTHFIEKYNHIHAAHVNIVCHRWTRMDIDGKPHPHSFIRDSEEKRNVQVDVVEGKGIDIKSSLSGLTVLKSTNSQFWGFLRDEYTTLKETWDRILSTDVDATWQWKNFSGLQEVRSHVPKFDATWATAREVTLKTFAEDNSASVQATMYKMAEQILARQQLIETVEYSLPNKHYFEIDLSWHKGLQNTGKNAEVFAPQSDPNGLIKCTVGRSXLKSKL

SEQ ID NO: 50 - protein, 301 aa, Artificial Sequence
  Asp.Uox Variant Subunit
SAVKAARYGKDNVRVYKVHKDEKTGVQTVYEMTVCVLLEGEIETSYXKADNSVIVATDSIKNTIYITAKQNPVTPPELFGSILGTHFIEKYNHIHAAHVNIVCHRWTRMDIDGKPHPHSFIRDSEEKRNVQVDVVEGKGIDIKSSLSGLTVLKSTNSQFWGFLRDEYTTLKETWDRILSTDVDATWQWKNFSGLQEVRSHVPKFDATWATAREVTLKTFAEDNSASVQATMYKMAEQILARQQLIETVEYSLPNKHYFEIDLSWHKGLQNTGKNAEVFAPQSDPNGLIKCTVGRSSLKSKL

SEQ ID NO: 51 - protein, 303 aa, Candida Utilis
MSTTLSSSTYGKDNVKFLKVKKDPQNPKKQEVMEATVTCLLEGGFDTSYTEADNSSIVPTDTVKNTILVLAKTTEIWPIERFAAKLATHFVEKYSHVSGVSVKIVQDRWVKYAVDGKPHDHSFIHEGGEKRITDLYYKRSGDYKLSSAIKDLTVLKSTGSMFYGYNKCDFTTLQPTTDRILSTDVDATWVWDNKKIGSVYDIAKAADKGIFDNVYNQAREITLTTFALENSPSVQATMFNMATQILEKACSVYSVSYALPNKHYFLIDLKWKGLENDNELFYPSPHPNGLIKCTVVRKEKTKL

SEQ ID NO: 52 - protein, 303 aa, Artificial Sequence
  Candida.Uox Variant Subunit
  MISC_FEATURE (1)..(303): Xaa is unnatural amino acid containing tetrazine functional group, and/or triazine functional group.
MSTTLSSSTYGKDNVKFLKVKKDPQNPKKQEVMEATVTCLLEGGFDTSYTEADNSSIVPTDTVKNTILVLAKTTEIWPIERFAAKLATHFVEKYSHVSGVSVKIVQDRWVKYAVDGKPHDHSFIHEGGEKRITDLYYKRSGDYKLSSAIKDLTVLKSTGSMFYGYNKCDFTTLQPTTDRILSTDVDATWVWDNKKIGSVYDIAKAADKGIFDNVYNQAREITLTTFALENSPSVQATMFNMATQILEKACSVYSVSYALPNKHYFLIDLKWKGLENDNELFYPSPHPNGLIKCTVVRKEKXKL

SEQ ID NO: 53 - protein, 303 aa, Artificial Sequence
  Candida.Uox Variant Subunit
MSTTLSSSTYGKDNVKFLKVKKDPQXPKKQEVMEATVTCLLEGGFDTSYTEADNSSIVPTDTVKNTILVLAKTTEIWPIERFAAKLATHFVEKYSHVSGVSVKIVQDRWVKYAVDGKPHDHSFIHEGGEKRITDLYYKRSGDYKLSSAIKDLTVLKSTGSMFYGYNKCDFTTLQPTTDRILSTDVDATWVWDNKKIGSVYDIAKAADKGIFDNVYNQAREITLTTFALENSPSVQATMFNMATQILEKACSVYSVSYALPNKHYFLIDLKWKGLENDNELFYPSPHPNGLIKCTVVRKEKTKL

SEQ ID NO: 54 - protein, 303 aa, Artificial Sequence
  Candida.Uox Variant Subunit
MSTTLSSSTYGKDNVKFLKVKKDPQNPKKQEVMEATVTCLLEGGFDTSYTEADNSSIVPTDTVKNTILVLAKTTEIWPIERFAAKLATHFVEKYSHVSGVSVKIVQDRWVKYAVDGKPHDHSFIHEGGEKRITDLYYKRSGDYKLSSAIKDLTVLKSTGSMFYGYNKCDFTTLQPTTDRILSTDVDATWVWDNKKIGSVYDIAKAADKGIFDNVYNQAREITLTTFALENSPSVQATMFNMATQILEKACSVYSVSYALPNKHYFLIDLKWKGLENDNELFYPSPHPNGLIKCTVVRKEKTKX

SEQ ID NO: 55 - protein, 303 aa, Artificial Sequence
  Candida.Uox Variant Subunit
  MISC_FEATURE (1)..(303): Xaa is unnatural amino acid containing tetrazine functional group, and/or triazine functional group.
MSTTLSSSTYGKDNVKFLKVKKDPQNPKKQEVMEATVTCLLEGGFDTSYTEADNSSIVPTDTVKNTILVLAKTTEIWPIERFAAKLATHFVEKYSHVSGVSVKIVQDRWVKYAVDGKPHDHSFIHEGGEKRITDLYYKRSGDYKLSSAIKDLTVLKSTGSMFYGYNKCDFTTLQPTTDRILSTDVDATWVWDNXKIGSVYDIAKAADKGIFDNVYNQAREITLTTFALENSPSVQATMFNMATQILEKACSVYSVSYALPNKHYFLIDLKWKGLENDNELFYPSPHPNGLIKCTVVRKEKTKL

SEQ ID NO: 56 - protein, 303 aa, Artificial Sequence
  Candida.Uox Variant Subunit
MSTTLSSSTYGKDNVKFLKVKKDPQNPKKQEVMEATVTCLLEGGFDTSYTEADNSSIVPTDTVKNTILVLAKTTEIWPIERFAAKLATHFVEKYXHVSGVSVKIVQDRWVKYAVDGKPHDHSFIHEGGEKRITDLYYKRSGDYKLSSAIKDLTVLKSTGSMFYGYNKCDFTTLQPTTDRILSTDVDATWVWDNKKIGSVYDIAKAADKGIFDNVYNQAREITLTTFALENSPSVQATMFNMATQILEKACSVYSVSYALPNKHYFLIDLKWKGLENDNELFYPSPHPNGLIKCTVVRKEKTKL

SEQ ID NO: 57 - protein, 303 aa, Artificial Sequence
  Candida.Uox Variant Subunit
  MISC_FEATURE (1)..(303): Xaa is unnatural amino acid containing tetrazine functional group, and/or triazine functional group.
MSTTLSSSTYGKDNVKFLKVKKDPQNPKKQEVMEATVTCLLEGGFDTSYTEADNSSIVPTDTVKNTILVLAKTTEIWPIERFAAKLATHFVEKYSHVSGVSVKIVQDRWVKYAVDGKPHDHSFIHEGGEKRITDLYYKRXGDYKLSSAIKDLTVLKSTGSMFYGYNKCDFTTLQPTTDRILSTDVDATWVWDNKKIGSVYDIAKAADKGIFDNVYNQAREITLTTFALENSPSVQATMFNMATQILEKACSVYSVSYALPNKHYFLIDLKWKGLENDNELFYPSPHPNGLIKCTVVRKEKTKL

SEQ ID NO: 58 - protein, 303 aa, Artificial Sequence
  Candida.Uox Variant Subunit
  MISC_FEATURE (1)..(303): Xaa is unnatural amino acid containing tetrazine functional group, and/or triazine functional group.
MSTTLSSSTYGKDNVKFLKVKKDPQNPKKQEVMEATVTCLLEGGFDTSYTEADNSSIVPTDTVKNTILVLAKTTEIWPIERFAAKLATHFVEKYSHVSGVSVKIVQDRWVKYAVDXKPHDHSFIHEGGEKRITDLYYKRSGDYKLSSAIKDLTVLKSTGSMFYGYNKCDFTTLQPTTDRILSTDVDATWVWDNKKIGSVYDIAKAADKGIFDNVYNQAREITLTTFALENSPSVQATMFNMATQILEKACSVYSVSYALPNKHYFLIDLKWKGLENDNELFYPSPHPNGLIKCTVVRKEKTKL

SEQ ID NO: 59 - protein, 303 aa, Artificial Sequence
  Candida.Uox Variant Subunit
  MISC_FEATURE (1)..(303): Xaa is unnatural amino acid containing tetrazine functional group, and/or triazine functional group.
MSTTLSSSTYGKDNVKFLKVKKDPQNPKKQEVMEATVTCLLEGGFDTSYTEADNSSIVPTDTVKNTILVLAKTTEIWPIERFAAKLATHFVEKYSHVSGVSVKIVQDRWVKYAVDGKPHDHSFIHEGGEKRITDLYYKRSGDYKLSSAIKDLTVLKSTGSMFYGYNKCDFTTLQPTTDRILSTDVDATWVWDNKKIGSVYDIAKAADKGIFDNVYNQAREITLTTFALENSPSVQATMFNMATQILEKACSVYSVSYALPNKHYFLIDLKWKGLENDNELFYPSPHPNGLIKCTVVRKEKTXL

SEQ ID NO: 60 - protein, 303 aa, Artificial Sequence
  Candida.Uox Variant Subunit
  MISC_FEATURE (1)..(303): Xaa is unnatural amino acid containing tetrazine functional group, and/or triazine functional group.
MSTTLSSSTYGKDNVKFLKVKKDPQNPKKQEVMEATVTCLLEGGFDTSYTEADNSSIVPTDTVKNTILVLAKTTEIWPIERFAAKLATHFVEKYSHVSGVSVKIVQDRWVKYAVDGKPHDHSFIHEGGEKRITDLYYKRSGDYKLSSAIKDLTVLKSTGSMFYGYNXCDFTTLQPTTDRILSTDVDATWVWDNKKIGSVYDIAKAADKGIFDNVYNQAREITLTTFALENSPSVQATMFNMATQILEKACSVYSVSYALPNKHYFLIDLKWKGLENDNELFYPSPHPNGLIKCTVVRKEKTKL

SEQ ID NO: 61 - protein, 303 aa, Artificial Sequence
  Candida.Uox Variant Subunit
  MISC_FEATURE (1)..(303): Xaa is unnatural amino acid containing tetrazine functional group, and/or triazine functional group.
MSTTLSSSTYGKDNVKFLKVKKDPQNPKKQEVMEATVTCLLEGGFDTSYTEADNSSIVPTDTVKNTILVLAKTTEIWPIERFAAKLATHFVEKYSHVSGVSVKIVQDRWVKYAVXGKPHDHSFIHEGGEKRITDLYYKRSGDYKLSSAIKDLTVLKSTGSMFYGYNKCDFTTLQPTTDRILSTDVDATWVWDNKKIGSVYDIAKAADKGIFDNVYNQAREITLTTFALENSPSVQATMFNMATQILEKACSVYSVSYALPNKHYFLIDLKWKGLENDNELFYPSPHPNGLIKCTVVRKEKTKL

SEQ ID NO: 62 - protein, 303 aa, Artificial Sequence
  Candida.Uox Variant Subunit
  MISC_FEATURE (1)..(303): Xaa is unnatural amino acid containing tetrazine functional group, and/or triazine functional group.
MSTTLSSSTYGKDNVKFLKVKKDPQNPKKQEVMEATVTCLLEGGFDTSYTEADNSSIVPTDTVKNTILVLAKTTEIWPIERFAAKLATHFVEKYSHVSGVSVKIVQDRWVKYAVDGKPHDHSFIHEGGEKRITDLYYKRSGDYKLSSAIKDLTVLKSTGSMFYGYNKCDFTTLQPTTDRILSTDVDATWVWDNKKIGSVYDIAKAADKGIFDNVYNQAREITLTTFALENSPSVQATMFNMATQILEKACSVYSVSYALPNKHYFLIDLKWKGLENDNELFYPSPHPNGLIKCTVVRKXKTKL

SEQ ID NO: 63 - protein, 303 aa, Artificial Sequence
  Candida.Uox Variant Subunit
  MISC_FEATURE (1)..(303): Xaa is unnatural amino acid containing tetrazine functional group, and/or triazine functional group.
MSTTLSSSTYGKDNVKFLKVKKDXQNPKKQEVMEATVTCLLEGGFDTSYTEADNSSIVPTDTVKNTILVLAKTTEIWPIERFAAKLATHFVEKYSHVSGVSVKIVQDRWVKYAVDGKPHDHSFIHEGGEKRITDLYYKRSGDYKLSSAIKDLTVLKSTGSMFYGYNKCDFTTLQPTTDRILSTDVDATWVWDNKKIGSVYDIAKAADKGIFDNVYNQAREITLTTFALENSPSVQATMFNMATQILEKACSVYSVSYALPNKHYFLIDLKWKGLENDNELFYPSPHPNGLIKCTVVRKEKTKL

SEQ ID NO: 64 - protein, 303 aa, Artificial Sequence
  Candida.Uox Variant Subunit
  MISC_FEATURE (1)..(303): Xaa is unnatural amino acid containing tetrazine functional group, and/or triazine functional group.
MSTTLSSSTYGKDNVKFLKVKKDPQNPKKQEVMEATVTCLLEGGFDTSYTEADNSSIVPTDTVKNTILVLAKTTEIWPIERFAAKLATHFVEKYSHVSGVSVKIVQDRWVKYAVDGKPHDHSFIHEGGEKRITDLYYKRSGDYKLSSAIKDLTVLKSTGSMFYGYNKCDFTTLQPTTDRILSTDVDATWVWDNKKIGSVYDIAKAADKGIFDNVYNQAREITLTTFALENSPSVQATMFNMATQILEKACSVYSVSYALPNKHYFLIDLKXKGLENDNELFYPSPHPNGLIKCTVVRKEKTKL

SEQ ID NO: 65 - protein, 303 aa, Artificial Sequence
  Candida.Uox Variant Subunit
  MISC_FEATURE (1)..(303): Xaa is unnatural amino acid containing tetrazine functional group, and/or triazine functional group.
MSTTLSSSTYGKDNVKFLKVKKDPQNPKKQEVMEATVTCLLEGGFDTSYTEADNSSIVPTDTVKNTILVLAKTTEIWPIERFAAKLATHFVEKYSHVSGVSVKIVQDRWVKYAVDGKPHDHSFIHEGGEKRITDLYYKRSGDYKLSSAIKDLTVLKSTGSMFYGYNKCDFTTLQPTTDRILSTDVDATWVWDNKKIGSVYDIAKAADKGIFDNVYNQAREITLTTFALENSPSVQATMFNMATQILEKACSVYSVSYALPNKHYFLIDLKWKGLENXNELFYPSPHPNGLIKCTVVRKEKTKL

SEQ ID NO: 66 - protein, 303 aa, Artificial Sequence
  Candida.Uox Variant Subunit
  MISC_FEATURE (1)..(303): Xaa is unnatural amino acid containing tetrazine functional group, and/or triazine functional group.
MSTTLSSSTYGKDNVKFLKVKKDPQNPKKQEVMEATVTCLLEGGFDTSYTEADNSSIVPTDTVKNTILVLAKTTEIWPIERFAAKLATHFVEKYSHVSGVSVKIVQDRWVKYAVDGKPHDHSFIHEGGEKRITDLYYKRSGDYKLSSAIKDLTVLKSTGSMFYGYNKCXFTTLQPTTDRILSTDVDATWVWDNKKIGSVYDIAKAADKGIFDNVYNQAREITLTTFALENSPSVQATMFNMATQILEKACSVYSVSYALPNKHYFLIDLKWKGLENDNELFYPSPHPNGLIKCTVVRKEKTKL

SEQ ID NO: 67 - protein, 303 aa, Artificial Sequence
  Candida.Uox Variant Subunit
  MISC_FEATURE (1)..(303): Xaa is unnatural amino acid containing tetrazine functional group, and/or triazine functional group.
MSTTLSSSTYGKDNVKFLKVKKDPQNPKKQEVMEATVTCLLEGGFDTSYTEADNSSIVPTDTVKNTILVLAKTTEIWPIERFAAKLATHFVEKYSHVSGVSVKIVQDRWVKYAVDGKXHDHSFIHEGGEKRITDLYYKRSGDYKLSSAIKDLTVLKSTGSMFYGYNKCDFTTLQPTTDRILSTDVDATWVWDNKKIGSVYDIAKAADKGIFDNVYNQAREITLTTFALENSPSVQATMFNMATQILEKACSVYSVSYALPNKHYFLIDLKWKGLENDNELFYPSPHPNGLIKCTVVRKEKTKL

SEQ ID NO: 68 - protein, 303 aa, Artificial Sequence
  Candida.Uox Variant Subunit
  MISC_FEATURE (1)..(303): Xaa is unnatural amino acid containing tetrazine functional group, and/or triazine functional group.
MSTTLSSSTYGKDNVKFLKVKKDPQNPKKQEVMEATVTCLLEGGFDTSYTEADNSSIVPTDTVKNTILVLAKTTEIWPIERFAAKLATHFVEKYSHVSGVSVKIVQDRWVKYAVDGKPHDHSFIHEGGEKRITDLYYKRSGDYKLSSAIKDLTVLKSTGSMFYGYNKCDFTTLQPTXDRILSTDVDATWVWDNKKIGSVYDIAKAADKGIFDNVYNQAREITLTTFALENSPSVQATMFNMATQILEKACSVYSVSYALPNKHYFLIDLKWKGLENDNELFYPSPHPNGLIKCTVVRKEKTKL

SEQ ID NO: 69 - protein, 303 aa, Artificial Sequence
  Candida.Uox Variant Subunit
  MISC_FEATURE (1)..(303): Xaa is unnatural amino acid containing tetrazine functional group, and/or triazine functional group.
MSTTLSSSTYGKDNVKFLKVKKDPQNPKKQEVMEATVTCLLEGGFDTSYTEADNSSIVPTDTVKNTILVLAKTTEIWPIERFAAKLATHFVEKYSHVSGVSVKIVQDRWVKYAVDGKPHDHSFIHEGGEKRITDLYYKRSGDYKLSSAIKDLTVLKSTGSMFYGYNKCDFTTLXPTTDRILSTDVDATWVWDNKKIGSVYDIAKAADKGIFDNVYNQAREITLTTFALENSPSVQATMFNMATQILEKACSVYSVSYALPNKHYFLIDLKWKGLENDNELFYPSPHPNGLIKCTVVRKEKTKL

SEQ ID NO: 70 - protein, 303 aa, Artificial Sequence
  Candida.Uox Variant Subunit
  MISC_FEATURE (1)..(303): Xaa is unnatural amino acid containing tetrazine functional group, and/or triazine functional group.
MSTTLSSSTYGKDNVKFLKVKKDPQNPKKQEVMEATVTCLLEGGFDTSYTEADNSSIVPTDTVKNTILVLAKTTEIWPIERFAAKLATHFVEKYSHVSGVSVKIVQDRWVKYAVDGKPHDHSFIHEGGEKRITDLYYKRSGDYKLSSAIKDLTVLKSTGSMFYGYNKCDFTTLQPTTDRILSTDVDATWVWDNKKIGSVYDIAKAADXGIFDNVYNQAREITLTTFALENSPSVQATMFNMATQILEKACSVYSVSYALPNKHYFLIDLKWKGLENDNELFYPSPHPNGLIKCTVVRKEKTKL

SEQ ID NO: 71 - protein, 303 aa, Artificial Sequence
  Candida.Uox Variant Subunit
  MISC_FEATURE (1)..(303): Xaa is unnatural amino acid containing tetrazine functional group, and/or triazine functional group.
MSTTLSSSTYGKDNVKFLKVKKDPQNPKKQEVMEATVTCLLEGGFDTSYTEADNSSIVPTDTVKNTILVLAKTTEIWPIERFAAKLATHFVEKYSHVSGVSVKIVQDRWVKYAVDGKPHDHSFIHEGGEKRITDLYYKRSGDYKLSSAIKDLTVLKSTGSMFYGYNKCDFTTLQPTTDRILSTDVDATWVWDNKKIGSVYDIAKAADKGIFDNVYNQAREITLTTFALENSPSVQATMFNMATQILEKACSVYSVSYALPNKHYFLIDLKWKGLXNDNELFYPSPHPNGLIKCTVVRKEKTKL

SEQ ID NO: 72 - protein, 303 aa, Artificial Sequence
  Candida.Uox Variant Subunit
  MISC_FEATURE (1)..(303): Xaa is unnatural amino acid containing tetrazine functional group, and/or triazine functional group.
MSTTLSSSTYGKDNVKFLKVKKDPQNPKKQEVMEATVTCLLEGGFDTSYTEADNSSIVPTDTVKNTILVLAKTTEIWPIERFAAKLATHFVEKYSHVSGVSVKIVQDRWVKYAVDGKPHDHSFIHEGGEKRITDLYYKRSGDYKLSSAIKDLTVLKSTGSMFYGYNKCDFTTLQPTTDRILSTDVDATWVWDNKKIGSVYDIAKAADKGIFDNVYNQAREITLTTFALENSPSVQATMFNMATQILEKACSVYSVSYALPNKHYFXIDLKWKGLENDNELFYPSPHPNGLIKCTVVRKEKTKL

SEQ ID NO: 73 - protein, 303 aa, Artificial Sequence
  Candida.Uox Variant Subunit
  MISC_FEATURE (1)..(303): Xaa is unnatural amino acid containing tetrazine functional group, and/or triazine functional group.
MSTTLSSSTYGKDNVKFLKVKKDPQNPKKQEVMEATVTCLLEGGFDTSYTEADNSSIVPTDTVKNTILVLAKTTEIWPIERFAAKLATHFVEKYSHVSGVSVKIVQDRWVKYAVDGKPHDHSFIHEGGEKRITDLYYKRSGDYKLSSAIKDLTVLKSTGSMFYGYNKCDFTTLQPTTDRILSTDVDATWVWDNKKIGSVYDIAKAADKGIFDNVYNQAREITLTTFALENSPSVQATMFNMATQILEKACSVYSVSYALPNKHYFLIDLKWKXLENDNELFYPSPHPNGLIKCTVVRKEKTKL

SEQ ID NO: 74 - protein, 303 aa, Artificial Sequence
  Candida.Uox Variant Subunit
  MISC_FEATURE (1)..(303): Xaa is unnatural amino acid containing tetrazine functional group, and/or triazine functional group.
MSTTLSSSTYGKDNVKFLKVKKDPQNPKKQEVMEATVTCLLEGGFDTSYTEADNSSIVPTDTVKNTILVLAKTTEIWPIERFAAKLATHFVEKYSHVSGVSVKIVQDRWVKYAVDGKPHDHSFIHEGGEKRITDLYYKRSGDYKLSSAIKDLTVLKSTGSMFYGYNKCDFTTLQPTTDRILSTDVDATWVWDNKKIGSVXDIAKAADKGIFDNVYNQAREITLTTFALENSPSVQATMFNMATQILEKACSVYSVSYALPNKHYFLIDLKWKGLENDNELFYPSPHPNGLIKCTVVRKEKTKL

SEQ ID NO: 75 - protein, 303 aa, Artificial Sequence
  Candida.Uox Variant Subunit
  MISC_FEATURE (1)..(303): Xaa is unnatural amino acid containing tetrazine functional group, and/or triazine functional group.
MSTTLSSSTYGKDNVKFLKVKKDPQNPKKQEVMEATVTCLLEGGFDTSYTEADNSSIVPTDTVKNTILVLAKTTEIWPIERFAAKLATHFVXKYSHVSGVSVKIVQDRWVKYAVDGKPHDHSFIHEGGEKRITDLYYKRSGDYKLSSAIKDLTVLKSTGSMFYGYNKCDFTTLQPTTDRILSTDVDATWVWDNKKIGSVYDIAKAADKGIFDNVYNQAREITLTTFALENSPSVQATMFNMATQILEKACSVYSVSYALPNKHYFLIDLKWKGLENDNELFYPSPHPNGLIKCTVVRKEKTKL

SEQ ID NO: 76 - protein, 303 aa, Artificial Sequence
  Candida.Uox Variant Subunit
  MISC_FEATURE (1)..(303): Xaa is unnatural amino acid containing tetrazine functional group, and/or triazine functional group.
MSTTLSSSTYGKDNVKFLKVKKDPQNPKKQEVMEATVTCLLEGGFDTSYTEADNSSIVPTDTVKNTILVLAKTTEIWPIERFAAKLATHFVEKYSHVSGVSVKIVQDRWVKYAVDGKPHDHSFIHEGGEKRITDLYYKRSGDYKLSSAIKDLTVLKSTGSMFYGYNKCDFTTLQPTTDRILSTDVDATWVWDNKKIGSVYDIAKAADKGIFDNVYNQAREITLTTFALENSPSVQATMFNMATQILXKACSVYSVSYALPNKHYFLIDLKWKGLENDNELFYPSPHPNGLIKCTVVRKEKTKL

SEQ ID NO: 77 - protein, 303 aa, Artificial Sequence
  Candida.Uox Variant Subunit
  MISC_FEATURE (1)..(303): Xaa is unnatural amino acid containing tetrazine functional group, and/or triazine functional group.
MSTTLSSSTYGKDNVKFLKVKKDPQNPKKQEVMEATVTCLLEGGFDTSYTEADNSSIVPTDTVKNTILVLAKTTEIWPIERFAAKLATHFVEKYSHVSGVSVKIVQDRWVKYAVDGKPHDHSFIHEGGEKRITDLYYKRSGDYKLSSAIKDLTVLKSTGSMFYGYNKCDFTTLQPTTDRILSTDVDATWVWDNKKIGSVYDIAKAADKGIFDNVYNQAREITLTTFAXENSPSVQATMFNMATQILEKACSVYSVSYALPNKHYFLIDLKWKGLENDNELFYPSPHPNGLIKCTVVRKEKTKL

SEQ ID NO: 78 - protein, 303 aa, Artificial Sequence
  Candida.Uox Variant Subunit
  MISC_FEATURE (1)..(303): Xaa is unnatural amino acid containing tetrazine functional group, and/or triazine functional group.
MSTTLSSSTYGKDNVKFLKVKKDPQNPKKQEVMEATVTCLLEGGFDTSYTEADNSSIVPTDTVKNTILVLAKTTEIWPIERFAAKLATHFVEKYSHVSGVSVKIVQDRWVKYAVDGKPHDHSFIHEGGEKRITDLYYKRSGDYKLSSAIKDLTVLKSTGSMFYGYNKCDFTTLQPTTDRILSTDVDATWVWDNKKIGSVYDIAKAADKGIFDNVYNQAREITLTTFALENSPSVQATMFNMATQILEKACSVYSVSYALPNKHYFLIDLKWKGLENDNELFYPSPHPNGLIKCTVVRKEXTKL

SEQ ID NO: 79 - protein, 303 aa, Artificial Sequence
  Candida.Uox Variant Subunit
  MISC_FEATURE (1)..(303): Xaa is unnatural amino acid containing tetrazine functional group, and/or triazine functional group.
MSTTLSSSTYGKDNVKFLKVKKDPQNPKKQEVMEATVTCLLEGGFDTSYTEADNSSIVPTDTVKNTILVLAKTTEIWPIERFAAKLATHFVEKYSHVSGVSVKIVQDRWVKYAVDGKPHDHSFIHEGGEKRITDLYYKRSGDYKLSSAIKDLTVLKSTGSMFYGYNKCDFTTLQPTTDRILSTDVDATWVWDNKKIGSVYDIAXAADKGIFDNVYNQAREITLTTFALENSPSVQATMFNMATQILEKACSVYSVSYALPNKHYFLIDLKWKGLENDNELFYPSPHPNGLIKCTVVRKEKTKL

SEQ ID NO: 80 - protein, 303 aa, Artificial Sequence
  Candida.Uox Variant Subunit
  MISC_FEATURE (1)..(303): Xaa is unnatural amino acid containing tetrazine functional group, and/or triazine functional group.
MSTTLSSSTYGKDNVKFLKVKKDPQNPKKQEVMEATVTCLLEGGFDTSYTXADNSSIVPTDTVKNTILVLAKTTEIWPIERFAAKLATHFVEKYSHVSGVSVKIVQDRWVKYAVDGKPHDHSFIHEGGEKRITDLYYKRSGDYKLSSAIKDLTVLKSTGSMFYGYNKCDFTTLQPTTDRILSTDVDATWVWDNKKIGSVYDIAKAADKGIFDNVYNQAREITLTTFALENSPSVQATMFNMATQILEKACSVYSVSYALPNKHYFLIDLKWKGLENDNELFYPSPHPNGLIKCTVVRKEKTKL

SEQ ID NO: 81 - protein, 303 aa, Artificial Sequence
  Candida.Uox Variant Subunit
  MISC_FEATURE (1)..(303): Xaa is unnatural amino acid containing tetrazine functional group, and/or triazine functional group.
MSTTLSSSTYGKDNVKFLKVKKDPQNPKKQEVMEATVTCLLEGGFDTSYTEADNSSIVPTDTVKNTILVLAKTTEIWPIERFAAKLATHFVEKYSHVSGVSVKIVQDRWVKYAVDGKPHDHSFIHEGGEKRITDLYYKRSGDYKLSSAIKDLTVLKSTGSMFYGYNKCDFTTLQPTTDRILSTDVDATWVWDNKKIGSVYDIAKAAXKGIFDNVYNQAREITLTTFALENSPSVQATMFNMATQILEKACSVYSVSYALPNKHYFLIDLKWKGLENDNELFYPSPHPNGLIKCTVVRKEKTKL

SEQ ID NO: 82 - protein, 303 aa, Artificial Sequence
  Candida.Uox Variant Subunit
  MISC_FEATURE (1)..(303): Xaa is unnatural amino acid containing tetrazine functional group, and/or triazine functional group.
MSTTLSSSTYGKDNVKFLKVKKDPQNPKKQEVMEATVTCLLEGGFDTSYTEADNSSIVPTDTVKNTILVLAKTTEIWPIERFAAKLATHFVEKYSHVSGVSVKIVQDRWVKYAVDGXPHDHSFIHEGGEKRITDLYYKRSGDYKLSSAIKDLTVLKSTGSMFYGYNKCDFTTLQPTTDRILSTDVDATWVWDNKKIGSVYDIAKAADKGIFDNVYNQAREITLTTFALENSPSVQATMFNMATQILEKACSVYSVSYALPNKHYFLIDLKWKGLENDNELFYPSPHPNGLIKCTVVRKEKTKL

SEQ ID NO: 83 - protein, 303 aa, Artificial Sequence
  Candida.Uox Variant Subunit
  MISC_FEATURE (1)..(303): Xaa is unnatural amino acid containing tetrazine functional group, and/or triazine functional group.
MSTTLSSSTYGKDNVKFLKVKKDPQNPKKQEVMEATVTCLLEGGFDTSYTEADNSSIVPTDTVKNTILVLAKTTEIWPIERFAAKLATHFVEKYSHVSGVSVKIVQDRWVKYAVDGKPHDHSFIHEGGEKRITDLYYKRSGDYKLSSAIKDLTVLKSTGSMFYGYNKCDFTTLQPTTDRILSTDVDATWVWDNKKIGSVYDIAKAADKGIFDNVYNQAREITLTTFALENSPSVQATMFNMATQILEKAXSVYSVSYALPNKHYFLIDLKWKGLENDNELFYPSPHPNGLIKCTVVRKEKTKL

SEQ ID NO: 84 - protein, 303 aa, Artificial Sequence
  Candida.Uox Variant Subunit
  MISC_FEATURE (1)..(303): Xaa is unnatural amino acid containing tetrazine functional group, and/or triazine functional group.
MSTTLSSSTYGKDNVKFLKVKKDPQNPKKQEVMEATVTCLLEGGFDTSYTEADNSSIVPTDTVKNTILVLAKTTEIWPIERFAAKLATHFVEKYSHVSGVSVKIVQDRWVKYAVDGKPHDHSFIHEGGEKRITDLYYKRSGDYKLSSAIKDLTVLKSTGSMFYGYNKCDFTTLQXTTDRILSTDVDATWVWDNKKIGSVYDIAKAADKGIFDNVYNQAREITLTTFALENSPSVQATMFNMATQILEKACSVYSVSYALPNKHYFLIDLKWKGLENDNELFYPSPHPNGLIKCTVVRKEKTKL

SEQ ID NO: 85 - protein, 303 aa, Artificial Sequence
  Candida.Uox Variant Subunit
  MISC_FEATURE (1)..(303): Xaa is unnatural amino acid containing tetrazine functional group, and/or triazine functional group.
MSTTLSSSTYGKDNVKFLKVKKDPQNPKKQEVMEATVTCLLEGGFDTSYTEADNSSIVPTDTVKNTILVLAKTTEIWPIERFAAKLATHFVEKYSHVSGVSVKIVQDRWVKYAVDGKPHDHSFIHEGGEKRITDLYYKRSGDYKLSSAIKDLTVLKSTGSMFYGYNKCDFTTLQPTTDRILSTDVDATWVWDNKKIGSVYDIAKAADKGIFDNVYNQAREITLTTFALENSPSVQATMFNMATQILEKACSVYSVSYALPNKHYFLIDLXWKGLENDNELFYPSPHPNGLIKCTVVRKEKTKL

SEQ ID NO: 86 - protein, 303 aa, Artificial Sequence
  Candida.Uox Variant Subunit
  MISC_FEATURE (1)..(303): Xaa is unnatural amino acid containing tetrazine functional group, and/or triazine functional group.
MSTTLSSSTYGKDNVKFLKVKKDPQNPKKQEVMEATVTCLLEGGFDTSYTEADNSSIVPTDTVKNTILVLAKTTEIWPIERFAAKLATHFVEKYSHVSGVSVKIVQDRWVKYAVDGKPHDHSFIHEGGEKRITDLYYKRSGDYKLSSAIKDLTVLKSTGSMFYGYNKCDFTTLQPTTDRILSTDVDATWVWDNKKIGSVYDIAKAADKGIFDNVYNQAREITLTTFALENSPSVQATMFNMATQILEKACSVYSVSYALPNKHYFLIXLKWKGLENDNELFYPSPHPNGLIKCTVVRKEKTKL

SEQ ID NO: 87 - protein, 303 aa, Artificial Sequence
  Candida.Uox Variant Subunit
  MISC_FEATURE (1)..(303): Xaa is unnatural amino acid containing tetrazine functional group, and/or triazine functional group.
MSTTLSSSTYGKDNVKFLKVKKDPQNPKKQEVMEATVTCLLEGXFDTSYTEADNSSIVPTDTVKNTILVLAKTTEIWPIERFAAKLATHFVEKYSHVSGVSVKIVQDRWVKYAVDGKPHDHSFIHEGGEKRITDLYYKRSGDYKLSSAIKDLTVLKSTGSMFYGYNKCDFTTLQPTTDRILSTDVDATWVWDNKKIGSVYDIAKAADKGIFDNVYNQAREITLTTFALENSPSVQATMFNMATQILEKACSVYSVSYALPNKHYFLIDLKWKGLENDNELFYPSPHPNGLIKCTVVRKEKTKL

SEQ ID NO: 88 - protein, 303 aa, Artificial Sequence
  Candida.Uox Variant Subunit
  MISC_FEATURE (1)..(303): Xaa is unnatural amino acid containing tetrazine functional group, and/or triazine functional group.
MSTTLSSSTYGKDNVKFLKVKKDPQNPKKQEVMEATVTCLLEGGFDTSYTEADNSSIVPTDTVKNTILVLAKTTEIWPIERFAAKLATHFVEKYSHVSGVSVKIVQDRWVKYAVDGKPHDHSFIHEGGEKRITDLYYKRSGDYKLSSAIKDLTVLKSTGSMFYGYNKCDFTTLQPTTDRILSTDVDATWVWDXKKIGSVYDIAKAADKGIFDNVYNQAREITLTTFALENSPSVQATMFNMATQILEKACSVYSVSYALPNKHYFLIDLKWKGLENDNELFYPSPHPNGLIKCTVVRKEKTKL

SEQ ID NO: 89 - protein, 303 aa, Artificial Sequence
  Candida.Uox Variant Subunit
  MISC_FEATURE (1)..(303): Xaa is unnatural amino acid containing tetrazine functional group, and/or triazine functional group.
MSTTLSSSTYGKDNVKFLKVKKDPQNPKKQEVMEATVTCLLEGGFDTSYTEADNSSIVPTDTVKNTILVLAKTTEIWPIERFAAKLATHFVEKYSHVSGVSVKIVQDRWVKYAVDGKPHDHSFIHEGGEKRITDLYYKRSGDYKLSSAIKDLTVLKSTGSMFYXYNKCDFTTLQPTTDRILSTDVDATWVWDNKKIGSVYDIAKAADKGIFDNVYNQAREITLTTFALENSPSVQATMFNMATQILEKACSVYSVSYALPNKHYFLIDLKWKGLENDNELFYPSPHPNGLIKCTVVRKEKTKL

SEQ ID NO: 90 - protein, 303 aa, Artificial Sequence
  Candida.Uox Variant Subunit
  MISC_FEATURE (1)..(303): Xaa is unnatural amino acid containing tetrazine functional group, and/or triazine functional group.
MSTTLSSSTYGKDNVKFLKVKKDPQNPKKQEVMEATVTCLLEGGFDTSYTEADNSSIVPTDTVKNTILVLAKXTEIWPIERFAAKLATHFVEKYSHVSGVSVKIVQDRWVKYAVDGKPHDHSFIHEGGEKRITDLYYKRSGDYKLSSAIKDLTVLKSTGSMFYGYNKCDFTTLQPTTDRILSTDVDATWVWDNKKIGSVYDIAKAADKGIFDNVYNQAREITLTTFALENSPSVQATMFNMATQILEKACSVYSVSYALPNKHYFLIDLKWKGLENDNELFYPSPHPNGLIKCTVVRKEKTKL

SEQ ID NO: 91 - protein, 303 aa, Artificial Sequence
  Candida.Uox Variant Subunit
  MISC_FEATURE (1)..(303): Xaa is unnatural amino acid containing tetrazine functional group, and/or triazine functional group.
MSTTLSSSTYGKDNVKFLKVKKDPQNPKXQEVMEATVTCLLEGGFDTSYTEADNSSIVPTDTVKNTILVLAKTTEIWPIERFAAKLATHFVEKYSHVSGVSVKIVQDRWVKYAVDGKPHDHSFIHEGGEKRITDLYYKRSGDYKLSSAIKDLTVLKSTGSMFYGYNKCDFTTLQPTTDRILSTDVDATWVWDNKKIGSVYDIAKAADKGIFDNVYNQAREITLTTFALENSPSVQATMFNMATQILEKACSVYSVSYALPNKHYFLIDLKWKGLENDNELFYPSPHPNGLIKCTVVRKEKTKL

SEQ ID NO: 92 - protein, 303 aa, Artificial Sequence
  Candida.Uox Variant Subunit
  MISC_FEATURE (1)..(303): Xaa is unnatural amino acid containing tetrazine functional group, and/or triazine functional group.
MSTTLSSSTYGKDNVKFLKVKKDPQNPKKQEVMEATVTCLLEGGFDTSYTEADNSSIVPTDTVKNTILVLAKTTEIWPIERFAAKLATHFVEKYSHVSGVSVKIVQDRWVKYAVDGKPHDHSFIHEGGEKRITDLYYKRSGDYKLSSAIKDLTVLKSTGSMFYGYNKCDFTTLQPTTDRILSTDVDATWVWDNKKIGSVYDIAKAADKGIFDNVYNQAREITLTTFALEXSPSVQATMFNMATQILEKACSVYSVSYALPNKHYFLIDLKWKGLENDNELFYPSPHPNGLIKCTVVRKEKTKL

SEQ ID NO: 93 - protein, 303 aa, Artificial Sequence
  Candida.Uox Variant Subunit
  MISC_FEATURE (1)..(303): Xaa is unnatural amino acid containing tetrazine functional group, and/or triazine functional group.
MSTTLSSSTYGKDNVKFLKVKKDPXNPKKQEVMEATVTCLLEGGFDTSYTEADNSSIVPTDTVKNTILVLAKTTEIWPIERFAAKLATHFVEKYSHVSGVSVKIVQDRWVKYAVDGKPHDHSFIHEGGEKRITDLYYKRSGDYKLSSAIKDLTVLKSTGSMFYGYNKCDFTTLQPTTDRILSTDVDATWVWDNKKIGSVYDIAKAADKGIFDNVYNQAREITLTTFALENSPSVQATMFNMATQILEKACSVYSVSYALPNKHYFLIDLKWKGLENDNELFYPSPHPNGLIKCTVVRKEKTKL

SEQ ID NO: 94 - protein, 303 aa, Artificial Sequence
  Candida.Uox Variant Subunit
  MISC_FEATURE (1)..(303): Xaa is unnatural amino acid containing tetrazine functional group, and/or triazine functional group.
MSTTLSSSTYGKDNVKFLKVKKDPQNPKKQEVMEATVTCLLEGGFDTSYTEADNSSIVPTDTVKNTILVLAKTTEIWPIERFAAKLATHFVEKYSHVSGVSVKIVQDRWVKYAVDGKPHDHSFIHEGGEKRITDLYYKRSGDYKLSSAIKDLTVLKSTGSMFYGYNKCDFTTLQPTTDRILSTDVDATWVWDNKKIGSVYDIAKAADKGIFDNVYXQAREITLTTFALENSPSVQATMFNMATQILEKACSVYSVSYALPNKHYFLIDLKWKGLENDNELFYPSPHPNGLIKCTVVRKEKTKL

SEQ ID NO: 95 - protein, 303 aa, Artificial Sequence
  Candida.Uox Variant Subunit
  MISC_FEATURE (1)..(303): Xaa is unnatural amino acid containing tetrazine functional group, and/or triazine functional group.
MSTTLSSSTYGKDNVKFLKVKKDPQNPKKQEVMEATVTCLLEGGFDTSYTEADNXSIVPTDTVKNTILVLAKTTEIWPIERFAAKLATHFVEKYSHVSGVSVKIVQDRWVKYAVDGKPHDHSFIHEGGEKRITDLYYKRSGDYKLSSAIKDLTVLKSTGSMFYGYNKCDFTTLQPTTDRILSTDVDATWVWDNKKIGSVYDIAKAADKGIFDNVYNQAREITLTTFALENSPSVQATMFNMATQILEKACSVYSVSYALPNKHYFLIDLKWKGLENDNELFYPSPHPNGLIKCTVVRKEKTKL

SEQ ID NO: 96 - protein, 303 aa, Artificial Sequence
  Candida.Uox Variant Subunit
  MISC_FEATURE (1)..(303): Xaa is unnatural amino acid containing tetrazine functional group, and/or triazine functional group.
MSTTLSSSTYGKDNVKFLKVKKDPQNPXKQEVMEATVTCLLEGGFDTSYTEADNSSIVPTDTVKNTILVLAKTTEIWPIERFAAKLATHFVEKYSHVSGVSVKIVQDRWVKYAVDGKPHDHSFIHEGGEKRITDLYYKRSGDYKLSSAIKDLTVLKSTGSMFYGYNKCDFTTLQPTTDRILSTDVDATWVWDNKKIGSVYDIAKAADKGIFDNVYNQAREITLTTFALENSPSVQATMFNMATQILEKACSVYSVSYALPNKHYFLIDLKWKGLENDNELFYPSPHPNGLIKCTVVRKEKTKL

SEQ ID NO: 97 - protein, 303 aa, Artificial Sequence
  Candida.Uox Variant Subunit
  MISC_FEATURE (1)..(303): Xaa is unnatural amino acid containing tetrazine functional group, and/or triazine functional group.
MSTTLXSSTYGKDNVKFLKVKKDPQNPKKQEVMEATVTCLLEGGFDTSYTEADNSSIVPTDTVKNTILVLAKTTEIWPIERFAAKLATHFVEKYSHVSGVSVKIVQDRWVKYAVDGKPHDHSFIHEGGEKRITDLYYKRSGDYKLSSAIKDLTVLKSTGSMFYGYNKCDFTTLQPTTDRILSTDVDATWVWDNKKIGSVYDIAKAADKGIFDNVYNQAREITLTTFALENSPSVQATMFNMATQILEKACSVYSVSYALPNKHYFLIDLKWKGLENDNELFYPSPHPNGLIKCTVVRKEKTKL

SEQ ID NO: 98 - protein, 303 aa, Artificial Sequence
  Candida.Uox Variant Subunit
  MISC_FEATURE (1)..(303): Xaa is unnatural amino acid containing tetrazine functional group, and/or triazine functional group.
MSTTLSSSTYGKDNVKFLKVKKDPQNXKKQEVMEATVTCLLEGGFDTSYTEADNSSIVPTDTVKNTILVLAKTTEIWPIERFAAKLATHFVEKYSHVSGVSVKIVQDRWVKYAVDGKPHDHSFIHEGGEKRITDLYYKRSGDYKLSSAIKDLTVLKSTGSMFYGYNKCDFTTLQPTTDRILSTDVDATWVWDNKKIGSVYDIAKAADKGIFDNVYNQAREITLTTFALENSPSVQATMFNMATQILEKACSVYSVSYALPNKHYFLIDLKWKGLENDNELFYPSPHPNGLIKCTVVRKEKTKL

SEQ ID NO: 99 - protein, 303 aa, Artificial Sequence
  Candida.Uox Variant Subunit
  MISC_FEATURE (1)..(303): Xaa is unnatural amino acid containing tetrazine functional group, and/or triazine functional group.
MSTTLSSSTYGKDNVKFLKVKKDPQNPKKQEVMEATVTCLLEGGFDTSYTEADNSSIVPTDTVKNTILVLAKTTEIWPIERFAAKLATHFVEKYSHVSGVSVKIVQDRWVKYAVDGKPHDHSFIHEGGEKRITDLYYKRSGDYKLSSAIKDLTVLKSTGSMFYGYNKCDFTTLQPTTDRILSTDVDATWVWDNKKIGSVYDIAKAADKGIFDNVYNQAREITLTTFALENSPSVQATMFNMATQILEKACSVYSVSYALPNKHYFLIDLKWKGLENDNELFYPSPHPNGLIKCTVVRXEKTKL

SEQ ID NO: 100 - protein, 303 aa, Artificial Sequence
  Candida.Uox Variant Subunit
  MISC_FEATURE (1)..(303): Xaa is unnatural amino acid containing tetrazine functional group, and/or triazine functional group.
MSTTLSSSTYGKDNVKFLKVKKDPQNPKKQEVMEATVTCLLEGGFDTSYTEADNSSIVPTDTVKNTILVLAKTTEIWPIERFAAKLATHFVEKYSHVSGVSVKIVQDRWVKYXVDGKPHDHSFIHEGGEKRITDLYYKRSGDYKLSSAIKDLTVLKSTGSMFYGYNKCDFTTLQPTTDRILSTDVDATWVWDNKKIGSVYDIAKAADKGIFDNVYNQAREITLTTFALENSPSVQATMFNMATQILEKACSVYSVSYALPNKHYFLIDLKWKGLENDNELFYPSPHPNGLIKCTVVRKEKTKL

SEQ ID NO: 101 - protein, 303 aa, Artificial Sequence
  Candida.Uox Variant Subunit
  MISC_FEATURE (1)..(303): Xaa is unnatural amino acid containing tetrazine functional group, and/or triazine functional group.
MSTTLSSSTYGKDNVKFLKVKKDPQNPKKQEVMEATVTCLLEGGFDTSYTEADNSSIVPTDTVKNTILVLAKTTEIWPIERFAAKLATHFVEKYSHVSGVSVKIVQDRWVKYAVDGKPHDHSFIHEGGEKRITDLYYKRSGDYKLSSAIKDLTVLKSTGSMFYGYNKCDFTTLQPTTDRILSTDVDATWVWDNKKIGSVYDIAKAADKGIFDXVYNQAREITLTTFALENSPSVQATMFNMATQILEKACSVYSVSYALPNKHYFLIDLKWKGLENDNELFYPSPHPNGLIKCTVVRKEKTKL

SEQ ID NO: 102 - protein, 303 aa, Artificial Sequence
  Candida.Uox Variant Subunit
  MISC_FEATURE (1)..(303): Xaa is unnatural amino acid containing tetrazine functional group, and/or triazine functional group.
MSTTLSSSTYGKDNVKFLKVKKDPQNPKKQEVMEATVTCLLEGGFDTSYTEADNSSIVPTDTVKNTILVLAKTTEIWPIERFAAKLATHFVEKYSHVSGVSVKIVQDRWVKYAVDGKPHDHSFIHEGGEKRITDLYYKRSGDYKLSSAIKDLTVLKSTGSMFYGYNKCDFTTLQPTTDRILSTDVDATWVWDNKKIGSVYDIAKAADKGIFDNVYNQARXITLTTFALENSPSVQATMFNMATQILEKACSVYSVSYALPNKHYFLIDLKWKGLENDNELFYPSPHPNGLIKCTVVRKEKTKL

SEQ ID NO: 103 - protein, 303 aa, Artificial Sequence
  Candida.Uox Variant Subunit
  MISC_FEATURE (1)..(303): Xaa is unnatural amino acid containing tetrazine functional group, and/or triazine functional group.
MSTTLSSSTYGKDNVKFLKVKKDPQNPKKQEVMEATVTCLLEGGFDTSYTEADNSSIVPTDTVKNTILVLAKTTEIWPIERFAAKLATHFVEKYSHVSGVSVKIVQDRWVKYAVDGKPHDHSFIHEGGEKRITDLYYKRSXDYKLSSAIKDLTVLKSTGSMFYGYNKCDFTTLQPTTDRILSTDVDATWVWDNKKIGSVYDIAKAADKGIFDNVYNQAREITLTTFALENSPSVQATMFNMATQILEKACSVYSVSYALPNKHYFLIDLKWKGLENDNELFYPSPHPNGLIKCTVVRKEKTKL

SEQ ID NO: 104 - protein, 303 aa, Artificial Sequence
  Candida.Uox Variant Subunit
  MISC_FEATURE (1)..(303): Xaa is unnatural amino acid containing tetrazine functional group, and/or triazine functional group.
MSTTLSSSTYGKDNVKFLKVKKDPQNPKKQEVMEATVTCLLEGGFDTSYTEADNSSIVPTDTVKNTILVLAKTTEIWPIERFAAKLATHFVEKYSHVSGVSVKIVQDRWVKYAVDGKPHDHSFIHEGGEKRITDLYYKRSGDYKLSSAIKDLTVLKSTGSMFXGYNKCDFTTLQPTTDRILSTDVDATWVWDNKKIGSVYDIAKAADKGIFDNVYNQAREITLTTFALENSPSVQATMFNMATQILEKACSVYSVSYALPNKHYFLIDLKWKGLENDNELFYPSPHPNGLIKCTVVRKEKTKL

SEQ ID NO: 105 - protein, 303 aa, Artificial Sequence
  Candida.Uox Variant Subunit
  MISC_FEATURE (1)..(303): Xaa is unnatural amino acid containing tetrazine functional group, and/or triazine functional group.
MSTTLSSSTYGKDNVKFLKVKKDPQNPKKQEVMEATVTCLLEGGFDTSYTEADNSSIVPTDTVKNTILVLAKTTEIWPIERFAAKLATHFVEKYSHVSGVSVKIVQDRWVKYAVDGKPHDHSFIHEGGEKRITDLYYKRSGDYKLSSAIKDLTVLKSTGSMFYGYNKCDFTTLQPTTDRILSTDVDATWVWDNKKIGSVYDIAKAADKGIFDNVYNQAREITLTTFALENSPSVQATMFNMATQILEKACSVXSVSYALPNKHYFLIDLKWKGLENDNELFYPSPHPNGLIKCTVVRKEKTKL

SEQ ID NO: 106 - protein, 303 aa, Artificial Sequence
  Candida.Uox Variant Subunit
  MISC_FEATURE (1)..(303): Xaa is unnatural amino acid containing tetrazine functional group, and/or triazine functional group.
MSTTLSSSTYGKDNVKFLKVKKDPQNPKKQEVMEATVTCLLEGGFDTSYTEADNSSIVPTDTVKNTILVLAKTTEIWPIERFAAKLATHFVEKYSHVSGVSVKIVQDRWVKYAVDGKPHDHSFIHEGGEKRITDLYYKRSGDYKLSSAIKDLTVLKSTGSMFYGYNKCDFTTLQPTTXRILSTDVDATWVWDNKKIGSVYDIAKAADKGIFDNVYNQAREITLTTFALENSPSVQATMFNMATQILEKACSVYSVSYALPNKHYFLIDLKWKGLENDNELFYPSPHPNGLIKCTVVRKEKTKL

SEQ ID NO: 107 - protein, 303 aa, Artificial Sequence
  Candida.Uox Variant Subunit
  MISC_FEATURE (1)..(303): Xaa is unnatural amino acid containing tetrazine functional group, and/or triazine functional group.
MSTTLSSSTYGKDNVKFLKVKKDPQNPKKQEVMEATVTCLLEGGFDTSYTEADNSSIVPTDTVKNTILVLAKTTEIWPIERFAAKLATHFVEXYSHVSGVSVKIVQDRWVKYAVDGKPHDHSFIHEGGEKRITDLYYKRSGDYKLSSAIKDLTVLKSTGSMFYGYNKCDFTTLQPTTDRILSTDVDATWVWDNKKIGSVYDIAKAADKGIFDNVYNQAREITLTTFALENSPSVQATMFNMATQILEKACSVYSVSYALPNKHYFLIDLKWKGLENDNELFYPSPHPNGLIKCTVVRKEKTKL

SEQ ID NO: 108 - protein, 303 aa, Artificial Sequence
  Candida.Uox Variant Subunit
  MISC_FEATURE (1)..(303): Xaa is unnatural amino acid containing tetrazine functional group, and/or triazine functional group.
MSTTLSSSTYGKDNVKFLKVKKDPQNPKKQEVMEATVTCLLEGGFDTSYTEADNSSIVPTDTVKNTILVLAKTTEIWPIERFAAKLATHFVEKYSHVSGVSVXIVQDRWVKYAVDGKPHDHSFIHEGGEKRITDLYYKRSGDYKLSSAIKDLTVLKSTGSMFYGYNKCDFTTLQPTTDRILSTDVDATWVWDNKKIGSVYDIAKAADKGIFDNVYNQAREITLTTFALENSPSVQATMFNMATQILEKACSVYSVSYALPNKHYFLIDLKWKGLENDNELFYPSPHPNGLIKCTVVRKEKTKL

SEQ ID NO: 109 - protein, 303 aa, Artificial Sequence
  Candida.Uox Variant Subunit
  MISC_FEATURE (1)..(303): Xaa is unnatural amino acid containing tetrazine functional group, and/or triazine functional group.
MSTTLSSSTYGKDNVKFLKVKKDPQNPKKQEVMEATVTCLLEGGFDTSYTEADNSSIVPTDTVKNTILVLAKTTEIWPIERFAAKLATHFVEKYSHVSGVSVKIVQDRWVKYAVDGKPHDHSFIHEGGEKRITDLYYKRSGDYXLSSAIKDLTVLKSTGSMFYGYNKCDFTTLQPTTDRILSTDVDATWVWDNKKIGSVYDIAKAADKGIFDNVYNQAREITLTTFALENSPSVQATMFNMATQILEKACSVYSVSYALPNKHYFLIDLKWKGLENDNELFYPSPHPNGLIKCTVVRKEKTKL

SEQ ID NO: 110 - protein, 303 aa, Artificial Sequence
  Candida.Uox Variant Subunit
  MISC_FEATURE (1)..(303): Xaa is unnatural amino acid containing tetrazine functional group, and/or triazine functional group.
MSTTLSSSTYGKDNVKFLKVKKDPQNPKKQEVMEATVTCLLEGGFDTSYTEADNSSIVPTDTVKNTILVLAKTTEIWPIERFAAKLATHFVEKYSHVSGVSVKIVQDRWVKYAVDGKPHDHSFIHEGGEKRITDLYYKXSGDYKLSSAIKDLTVLKSTGSMFYGYNKCDFTTLQPTTDRILSTDVDATWVWDNKKIGSVYDIAKAADKGIFDNVYNQAREITLTTFALENSPSVQATMFNMATQILEKACSVYSVSYALPNKHYFLIDLKWKGLENDNELFYPSPHPNGLIKCTVVRKEKTKL

SEQ ID NO: 111 - protein, 303 aa, Artificial Sequence
  Candida.Uox Variant Subunit
  MISC_FEATURE (1)..(303): Xaa is unnatural amino acid containing tetrazine functional group, and/or triazine functional group.
MSTTLSSSTYGKDNVKFLKVKKDPQNPKKQEVMEATVTCLLEGGFDTSYTEADNSSIVPTDTVKNTILVLAKTTEIWPIERFAAKLATHFVEKYSHVSGVSVKIVQDRWVKYAVDGKPHDHSFIHEGGEKRITDLYYXRSGDYKLSSAIKDLTVLKSTGSMFYGYNKCDFTTLQPTTDRILSTDVDATWVWDNKKIGSVYDIAKAADKGIFDNVYNQAREITLTTFALENSPSVQATMFNMATQILEKACSVYSVSYALPNKHYFLIDLKWKGLENDNELFYPSPHPNGLIKCTVVRKEKTKL

SEQ ID NO: 112 - protein, 303 aa, Artificial Sequence
  Candida.Uox Variant Subunit
  MISC_FEATURE (1)..(303): Xaa is unnatural amino acid containing tetrazine functional group, and/or triazine functional group.
MSTTLSXSTYGKDNVKFLKVKKDPQNPKKQEVMEATVTCLLEGGFDTSYTEADNSSIVPTDTVKNTILVLAKTTEIWPIERFAAKLATHFVEKYSHVSGVSVKIVQDRWVKYAVDGKPHDHSFIHEGGEKRITDLYYKRSGDYKLSSAIKDLTVLKSTGSMFYGYNKCDFTTLQPTTDRILSTDVDATWVWDNKKIGSVYDIAKAADKGIFDNVYNQAREITLTTFALENSPSVQATMFNMATQILEKACSVYSVSYALPNKHYFLIDLKWKGLENDNELFYPSPHPNGLIKCTVVRKEKTKL

SEQ ID NO: 113 - protein, 303 aa, Artificial Sequence
  Candida.Uox Variant Subunit
  MISC_FEATURE (1)..(303): Xaa is unnatural amino acid containing tetrazine functional group, and/or triazine functional group.
MSTTLSSSTYGKDNVKFLKVKKDPQNPKKQEVMEATVTCLLEGGFDTSYTEADNSSIVPTDTVKNTILVLAKTTEIWPIERFAAKLATHFVEKYSHVSGVSVKIVQDRWVKYAVDGKPHDHSFIHEGGEKRITDLYYKRSGDYKLSSAIKXLTVLKSTGSMFYGYNKCDFTTLQPTTDRILSTDVDATWVWDNKKIGSVYDIAKAADKGIFDNVYNQAREITLTTFALENSPSVQATMFNMATQILEKACSVYSVSYALPNKHYFLIDLKWKGLENDNELFYPSPHPNGLIKCTVVRKEKTKL

SEQ ID NO: 114 - protein, 303 aa, Artificial Sequence
  Candida.Uox Variant Subunit
  MISC_FEATURE (1)..(303): Xaa is unnatural amino acid containing tetrazine functional group, and/or triazine functional group.
MSTTLSSSTYGKDNVKFLKVKKDPQNPKKQEVMEATVTCLLEGGFDTSYTEADNSSIVPTDTVKNTILVLAKTTEIWPIERFAAKLATHFVEKYSHVSGVSVKIVQDRWVKYAVDGKPHDHSFIHEGGEKRITDLYYKRSGDYKLSSAIKDLTVLKSTGSMFYGYNKCDFTTLQPTTDRILSTDVDATWVWDNKKIGSVYDIAKAADKGIFDNVYNQAREITLTTFALENSPSVQATMFNMATQILEKACSVYSVSYALPNKHYFLIDLKWKGLENDNELFYPSPHPNGLIKCTVVXKEKTKL

SEQ ID NO: 115 - protein, 303 aa, Artificial Sequence
  Candida.Uox Variant Subunit
  MISC_FEATURE (1)..(303): Xaa is unnatural amino acid containing tetrazine functional group, and/or triazine functional group.
MSTTLSSSTYGKDNVKFLKVKKDPQNPKKQEVMEATVTCLLEGGFDTSYTEADNSSIVPTDTVKNTILVLAKTTEIWPIERFAAKLATHFVEKYSHVSGVSVKIVQDRWVKYAVDGKPHDHSFIHEGGEKRITDLYYKRSGDYKLSSAIKDLTVLKSTGSMFYGYNKCDFTTLQPTTDRILSTDVDATWVWDNKKIGSVYDIAKAADKGIFDNVYNQAREITLTTFALENSPSVQATMFNMATQILEKACSVYSVSYALPNKHYFLIDLKWXGLENDNELFYPSPHPNGLIKCTVVRKEKTKL

SEQ ID NO: 116 - protein, 303 aa, Artificial Sequence
  Candida.Uox Variant Subunit
  MISC_FEATURE (1)..(303): Xaa is unnatural amino acid containing tetrazine functional group, and/or triazine functional group.
MSTTLSSSTYGKDNVKFLKVKKDPQNPKKQEVMEATVTCLLEGGFDTSYTEADNSSIVPTDTVKNTILVLAKTTEIWPIERFAAKLATHFVEKYSHVSGVSVKIVQDRWVKYAVDGKPHDHSFIHEGGEKRITDLYYKRSGDYKLSSAIKDLTVLKSTGSMFYGYNKCDFTTLQPTTDRILSTDVDATWVWDNKKIGSVYDIAKAADKGIFDNVYNQAREITLTTFALENSPSVQATMFNMATQILEKACSVYSVSYALPNKHYFLIDLKWKGLENDXELFYPSPHPNGLIKCTVVRKEKTKL

SEQ ID NO: 117 - protein, 303 aa, Artificial Sequence
  Candida.Uox Variant Subunit
  MISC_FEATURE (1)..(303): Xaa is unnatural amino acid containing tetrazine functional group, and/or triazine functional group.
MSTTLSSSTYGKDNVKFLKVKKDPQNPKKQEVMEATVTCLLEGGFDTSYTEADNSSIVPTDTVKNTILVLAKTTEIWPIERFAAKLATHFVEKYSHVSGVSVKIVQDRWVKYAVDGKPHDHSFIHEGGEKRITDLYYKRSGDYKLSSAIKDLTVLKSTGSMFYGYNKCDFTTLQPTTDRILSTDVDATWVWDNKKIGSVYDIAKAADKGIFDNVYNQAREITLTTFALENSPSVQATMFNMATQILEKACSVYSVSYALPNKHYXLIDLKWKGLENDNELFYPSPHPNGLIKCTVVRKEKTKL

SEQ ID NO: 118 - protein, 302 aa, Arthrobacter Globiformis
MTATAETSTGTKVVLGQNQYGKAEVRLVKVTRNTARHEIQDLNVTSQLRGDFEAAHTAGDNAHVVATDTQKNTVYAFARDGFATTEEFLLRLGKHFTEGFDWVTGGRWAAQQFFWDRINDHDHAFSRNKSEVRTAVLEISGSEQAIVAGIEGLTVLKSTGSEFHGFPRDKYTTLQETTDRILATDVSARWRYNTVEVDFDAVYASVRGLLLKAFAETHSLALQQTMYEMGRAVIETHPEIDEIKMSLPNKHHFLVDLQPFGQDNPNEVFYAADRPYGLIEATIQREGSRADHPIWSNIAGFC

SEQ ID NO: 119 - protein, 302 aa, Artificial Sequence
  Arth.Uox Variant Subunit
  MISC_FEATURE (1)..(302): Xaa is unnatural amino acid containing tetrazine functional group, and/or triazine functional group.
MTATAETSTGTKVVLGQNQYGKAEVRLVKVTRNTARHEIQDLNVTSQLRGDFEAAHTAGDNAHVVATDTQKNTVYAFARXGFATTEEFLLRLGKHFTEGFDWVTGGRWAAQQFFWDRINDHDHAFSRNKSEVRTAVLEISGSEQAIVAGIEGLTVLKSTGSEFHGFPRDKYTTLQETTDRILATDVSARWRYNTVEVDFDAVYASVRGLLLKAFAETHSLALQQTMYEMGRAVIETHPEIDEIKMSLPNKHHFLVDLQPFGQDNPNEVFYAADRPYGLIEATIQREGSRADHPIWSNIAGFC

SEQ ID NO: 120 - protein, 302 aa, Artificial Sequence
  Arth.Uox Variant Subunit
  MISC_FEATURE (1)..(302): Xaa is unnatural amino acid containing tetrazine functional group, and/or triazine functional group.
MTATAETSTGTKVVLGQNQYGKAEVRLVKVTRNTARHEIQDLNVTSQLRGDFEAAHTAGDNAHVVATDTQKNTVYAFARDGXATTEEFLLRLGKHFTEGFDWVTGGRWAAQQFFWDRINDHDHAFSRNKSEVRTAVLEISGSEQAIVAGIEGLTVLKSTGSEFHGFPRDKYTTLQETTDRILATDVSARWRYNTVEVDFDAVYASVRGLLLKAFAETHSLALQQTMYEMGRAVIETHPEIDEIKMSLPNKHHFLVDLQPFGQDNPNEVFYAADRPYGLIEATIQREGSRADHPIWSNIAGFC

SEQ ID NO: 121 - protein, 302 aa, Artificial Sequence
  Arth.Uox Variant Subunit
  MISC_FEATURE (1)..(302): Xaa is unnatural amino acid containing tetrazine functional group, and/or triazine functional group.
MTATAETSTGTKVVLGQNQYGKAEVRLVKVTRNTARHEIQDLNVTSQLRGDFEAAHTAGDNAHVVATDTQKNTVYAFARDGFATTEEFLLRLGKHFTEGXDWVTGGRWAAQQFFWDRINDHDHAFSRNKSEVRTAVLEISGSEQAIVAGIEGLTVLKSTGSEFHGFPRDKYTTLQETTDRILATDVSARWRYNTVEVDFDAVYASVRGLLLKAFAETHSLALQQTMYEMGRAVIETHPEIDEIKMSLPNKHHFLVDLQPFGQDNPNEVFYAADRPYGLIEATIQREGSRADHPIWSNIAGFC

SEQ ID NO: 122 - protein, 302 aa, Artificial Sequence
  Arth.Uox Variant Subunit
  MISC_FEATURE (1)..(302): Xaa is unnatural amino acid containing tetrazine functional group, and/or triazine functional group.
MTATAETSTGTKVVLGQNQYGKAEVRLVKVTRNTARHEIQDLNVTSQLRGDFEAAHTAGDNAHVVATDTQKNTVYAFARDGFATTEEFLLRLGKHFTEGFXWVTGGRWAAQQFFWDRINDHDHAFSRNKSEVRTAVLEISGSEQAIVAGIEGLTVLKSTGSEFHGFPRDKYTTLQETTDRILATDVSARWRYNTVEVDFDAVYASVRGLLLKAFAETHSLALQQTMYEMGRAVIETHPEIDEIKMSLPNKHHFLVDLQPFGQDNPNEVFYAADRPYGLIEATIQREGSRADHPIWSNIAGFC

SEQ ID NO: 123 - protein, 302 aa, Artificial Sequence
  Arth.Uox Variant Subunit
  MISC_FEATURE (1)..(302): Xaa is unnatural amino acid containing tetrazine functional group, and/or triazine functional group.
MTATAETSTGTKVVLGQNQYGKAEVRLVKVTRNTARHEIQDLNVTSQLRGDFEAAHTAGDNAHVVATDTQKNTVYAFARDGFATTEEFLLRLGKHFTEGFDWVTGGRWAAQQFXWDRINDHDHAFSRNKSEVRTAVLEISGSEQAIVAGIEGLTVLKSTGSEFHGFPRDKYTTLQETTDRILATDVSARWRYNTVEVDFDAVYASVRGLLLKAFAETHSLALQQTMYEMGRAVIETHPEIDEIKMSLPNKHHFLVDLQPFGQDNPNEVFYAADRPYGLIEATIQREGSRADHPIWSNIAGFC

SEQ ID NO: 124 - protein, 302 aa, Artificial Sequence
  Arth.Uox Variant Subunit
  MISC_FEATURE (1)..(302): Xaa is unnatural amino acid containing tetrazine functional group, and/or triazine functional group.
MTATAETSTGTKVVLGQNQYGKAEVRLVKVTRNTARHEIQDLNVTSQLRGDFEAAHTAGDNAHVVATDTQKNTVYAFARDGFATTEEFLLRLGKHFTEGFDWVTGGRWAAQQFFWDRIXDHDHAFSRNKSEVRTAVLEISGSEQAIVAGIEGLTVLKSTGSEFHGFPRDKYTTLQETTDRILATDVSARWRYNTVEVDFDAVYASVRGLLLKAFAETHSLALQQTMYEMGRAVIETHPEIDEIKMSLPNKHHFLVDLQPFGQDNPNEVFYAADRPYGLIEATIQREGSRADHPIWSNIAGFC

SEQ ID NO: 125 - protein, 302 aa, Artificial Sequence
  Arth.Uox Variant Subunit
  MISC_FEATURE (1)..(302): Xaa is unnatural amino acid containing tetrazine functional group, and/or triazine functional group.
MTATAETSTGTKVVLGQNQYGKAEVRLVKVTRNTARHEIQDLNVTSQLRGDFEAAHTAGDNAHVVATDTQKNTVYAFARDGFATTEEFLLRLGKHFTEGFDWVTGGRWAAQQFFWDRINXHDHAFSRNKSEVRTAVLEISGSEQAIVAGIEGLTVLKSTGSEFHGFPRDKYTTLQETTDRILATDVSARWRYNTVEVDFDAVYASVRGLLLKAFAETHSLALQQTMYEMGRAVIETHPEIDEIKMSLPNKHHFLVDLQPFGQDNPNEVFYAADRPYGLIEATIQREGSRADHPIWSNIAGFC

SEQ ID NO: 126 - protein, 302 aa, Artificial Sequence
  Arth.Uox Variant Subunit
  MISC_FEATURE (1)..(302): Xaa is unnatural amino acid containing tetrazine functional group, and/or triazine functional group.
MTATAETSTGTKVVLGQNQYGKAEVRLVKVTRNTARHEIQDLNVTSQLRGDFEAAHTAGDNAHVVATDTQKNTVYAFARDGFATTEEFLLRLGKHFTEGFDWVTGGRWAAQQFFWDRINDHDHAFSRNKSEVRTAVLEISGXEQAIVAGIEGLTVLKSTGSEFHGFPRDKYTTLQETTDRILATDVSARWRYNTVEVDFDAVYASVRGLLLKAFAETHSLALQQTMYEMGRAVIETHPEIDEIKMSLPNKHHFLVDLQPFGQDNPNEVFYAADRPYGLIEATIQREGSRADHPIWSNIAGFC

SEQ ID NO: 127 - protein, 302 aa, Artificial Sequence
  Arth.Uox Variant Subunit
  MISC_FEATURE (1)..(302): Xaa is unnatural amino acid containing tetrazine functional group, and/or triazine functional group.
MTATAETSTGTKVVLGQNQYGKAEVRLVKVTRNTARHEIQDLNVTSQLRGDFEAAHTAGDNAHVVATDTQKNTVYAFARDGFATTEEFLLRLGKHFTEGFDWVTGGRWAAQQFFWDRINDHDHAFSRNKSEVRTAVLEISGSXQAIVAGIEGLTVLKSTGSEFHGFPRDKYTTLQETTDRILATDVSARWRYNTVEVDFDAVYASVRGLLLKAFAETHSLALQQTMYEMGRAVIETHPEIDEIKMSLPNKHHFLVDLQPFGQDNPNEVFYAADRPYGLIEATIQREGSRADHPIWSNIAGFC

SEQ ID NO: 128 - protein, 302 aa, Artificial Sequence
  Arth.Uox Variant Subunit
  MISC_FEATURE (1)..(302): Xaa is unnatural amino acid containing tetrazine functional group, and/or triazine functional group.
MTATAETSTGTKVVLGQNQYGKAEVRLVKVTRNTARHEIQDLNVTSQLRGDFEAAHTAGDNAHVVATDTQKNTVYAFARDGFATTEEFLLRLGKHFTEGFDWVTGGRWAAQQFFWDRINDHDHAFSRNKSEVRTAVLEISGSEQAIVAGIEGLTVLKSTGSEFHGFPRDKYTTLXETTDRILATDVSARWRYNTVEVDFDAVYASVRGLLLKAFAETHSLALQQTMYEMGRAVIETHPEIDEIKMSLPNKHHFLVDLQPFGQDNPNEVFYAADRPYGLIEATIQREGSRADHPIWSNIAGFC

SEQ ID NO: 129 - protein, 302 aa, Artificial Sequence
  Arth.Uox Variant Subunit
  MISC_FEATURE (1)..(302): Xaa is unnatural amino acid containing tetrazine functional group, and/or triazine functional group.
MTATAETSTGTKVVLGQNQYGKAEVRLVKVTRNTARHEIQDLNVTSQLRGDFEAAHTAGDNAHVVATDTQKNTVYAFARDGFATTEEFLLRLGKHFTEGFDWVTGGRWAAQQFFWDRINDHDHAFSRNKSEVRTAVLEISGSEQAIVAGIEGLTVLKSTGSEFHGFPRDKYTTLQETTDRILATDVSARWRYNTXEVDFDAVYASVRGLLLKAFAETHSLALQQTMYEMGRAVIETHPEIDEIKMSLPNKHHFLVDLQPFGQDNPNEVFYAADRPYGLIEATIQREGSRADHPIWSNIAGFC

SEQ ID NO: 130 - protein, 302 aa, Artificial Sequence
  Arth.Uox Variant Subunit
  MISC_FEATURE (1)..(302): Xaa is unnatural amino acid containing tetrazine functional group, and/or triazine functional group.
MTATAETSTGTKVVLGQNQYGKAEVRLVKVTRNTARHEIQDLNVTSQLRGDFEAAHTAGDNAHVVATDTQKNTVYAFARDGFATTEEFLLRLGKHFTEGFDWVTGGRWAAQQFFWDRINDHDHAFSRNKSEVRTAVLEISGSEQAIVAGIEGLTVLKSTGSEFHGFPRDKYTTLQETTDRILATDVSARWRYNTVXVDFDAVYASVRGLLLKAFAETHSLALQQTMYEMGRAVIETHPEIDEIKMSLPNKHHFLVDLQPFGQDNPNEVFYAADRPYGLIEATIQREGSRADHPIWSNIAGFC

SEQ ID NO: 131 - protein, 302 aa, Artificial Sequence
  Arth.Uox Variant Subunit
  MISC_FEATURE (1)..(302): Xaa is unnatural amino acid containing tetrazine functional group, and/or triazine functional group.
MTATAETSTGTKVVLGQNQYGKAEVRLVKVTRNTARHEIQDLNVTSQLRGDFEAAHTAGDNAHVVATDTQKNTVYAFARDGFATTEEFLLRLGKHFTEGFDWVTGGRWAAQQFFWDRINDHDHAFSRNKSEVRTAVLEISGSEQAIVAGIEGLTVLKSTGSEFHGFPRDKYTTLQETTDRILATDVSARWRYNTVEVDFDAVYASVRGLLLKAFAETXSLALQQTMYEMGRAVIETHPEIDEIKMSLPNKHHFLVDLQPFGQDNPNEVFYAADRPYGLIEATIQREGSRADHPIWSNIAGFC

SEQ ID NO: 132 - protein, 302 aa, Artificial Sequence
  Arth.Uox Variant Subunit
  MISC_FEATURE (1)..(302): Xaa is unnatural amino acid containing tetrazine functional group, and/or triazine functional group.
MTATAETSTGTKVVLGQNQYGKAEVRLVKVTRNTARHEIQDLNVTSQLRGDFEAAHTAGDNAHVVATDTQKNTVYAFARDGFATTEEFLLRLGKHFTEGFDWVTGGRWAAQQFFWDRINDHDHAFSRNKSEVRTAVLEISGSEQAIVAGIEGLTVLKSTGSEFHGFPRDKYTTLQETTDRILATDVSARWRYNTVEVDFDAVYASVRGLLLKAFAETHSLALQQTMYEMGRAVIETHXEIDEIKMSLPNKHHFLVDLQPFGQDNPNEVFYAADRPYGLIEATIQREGSRADHPIWSNIAGFC

SEQ ID NO: 133 - protein, 585 aa, Homo sapiens [sequence omitted]

SEQ ID NO: 134 - protein, 585 aa, Artificial Sequence
  Human Serum Albumin Variant
DAHKSEVAHRFKDLGEENFKALVLIAFAQYLQQCPFEDHVKLVNEVTEFAKTCVADESAENCDKSLHTLFGDKLCTVATLRETYGEMADCCAKQEPERNECFLQHKDDNPNLPRLVRPEVDVMCTAFHDNEETFLKKYLYEIARRHPYFYAPELLFFAKRYKAAFTECCQAADKAACLLPKLDELRDEGKASSAKQRLKCASLQKFGERAFKAWAVARLSQRFPKAEFAEVSKLVTDLTKVHTECCHGDLLECADDRADLAKYICENQDSISSKLKECCEKPLLEKSHCIAEVENDEMPADLPSLAADFVESKDVCKNYAEAKDVFLGMFLYEYARRHPDYSVVLLLRLAKTYETTLEKCCAAADPHECYAKVFDEFKPLVEEPQNLIKQNCELFEQLGEYKFQNALLVRYTKKVPQMSTPTLVEVSRNLGKVGSKCCKHPEAKRMPCAEDYLSVVLNQLCVLHEKTPVSDRVTKCCTESLVNRRPCFSALEVDETYVPKEFNAETFTFHADICTLSEKERQIKKQTALVELVKHKPKATKEQLKAVMDDFAAFVEKCCKADDKETCFAEEGKKLVAASQAALGL

SEQ ID NO: 135 - protein, 585 aa, Artificial Sequence
  Human Serum Albumin Variant
DAHKSEVAHRFKDLGEENFKALVLIAFAQYLQQCPFEDHVKLVNEVTEFAKTCVADESAENCDKSLHTLFGDKLCTVATLRETYGEMADCCAKQEPERNECFLQHKDDNPNLPRLVRPEVDVMCTAFHDNEETFLKKYLYEIARRHPYFYAPELLFFAKRYKAAFTECCQAADKAACLLPKLDELRDEGKASSAKQRLKCASLQKFGERAFKAWAVARLSQRFPKAEFAEVSKLVTDLTKVHTECCHGDLLECADDRADLAKYICENQDSISSKLKECCEKPLLEKSHCIAEVENDEMPADLPSLAADFVESKDVCKNYAEAKDVFLGMFLYEYARRHPDYSVVLLLRLAKTYETTLEKCCAAADPHECYAKVFDEFKPLVEEPQNLIKQNCELFEQLGEYKFQNALLVRYTKKVPQVSAPTLVEVSRNLGKVGSKCCKHPEAKRMPCAEDYLSVVLNQLCVLHEKTPVSDRVTKCCTESLVNRRPCFSALEVDETYVPKEFNAETFTFHADICTLSEKERQIKKQTALVELVKHKPKATKEQLKAVMDDFAAFVEKCCKADDKETCFAEEGKKLVAASQAALGL

SEQ ID NO: 136 - protein, 585 aa, Artificial Sequence
  Human Serum Albumin Variant
DAHKSEVAHRFKDLGEENFKALVLIAFAQYLQQCPFEDHVKLVNEVTEFAKTCVADESAENCDKSLHTLFGDKLCTVATLRETYGEMADCCAKQEPERNECFLQHKDDNPNLPRLVRPEVDVMCTAFHDNEETFLKKYLYEIARRHPYFYAPELLFFAKRYKAAFTECCQAADKAACLLPKLDELRDEGKASSAKQRLKCASLQKFGERAFKAWAVARLSQRFPKAEFAEVSKLVTDLTKVHTECCHGDLLECADDRADLAKYICENQDSISSKLKECCEKPLLEKSHCIAEVENDEMPADLPSLAADFVESKDVCKNYAEAKDVFLGMFLYEYARRHPDYSVVLLLRLAKTYETTLEKCCAAADPHECYAKVFDEFKPLVEEPQNLIKQNCELFEQLGEYKFQNALLVRYTKKVPQVSTPTLVEVSRNLGKVGSKCCKHPEAKRMPCAEDYLSVVLNQLCVLHEKTPVSDRVTKCCTESLVNRRPCFSALEVDETYVPKEFNARTFTFHADICTLSEKERQIKKQTALVELVKHKPKATKEQLKAVMDDFAAFVEKCCKADDKETCFAEEGKKLVAASQAALGL

SEQ ID NO: 137 - protein, 585 aa, Artificial Sequence
  Human Serum Albumin Variant
DAHKSEVAHRFKDLGEENFKALVLIAFAQYLQQCPFEDHVKLVNEVTEFAKTCVADESAENCDKSLHTLFGDKLCTVATLRETYGEMADCCAKQEPERNECFLQHKDDNPNLPRLVRPEVDVMCTAFHDNEETFLKKYLYEIARRHPYFYAPELLFFAKRYKAAFTECCQAADKAACLLPKLDELRDEGKASSAKQRLKCASLQKFGERAFKAWAVARLSQRFPKAEFAEVSKLVTDLTKVHTECCHGDLLECADDRADLAKYICENQDSISSKLKECCEKPLLEKSHCIAEVENDEMPADLPSLAADFVESKDVCKNYAEAKDVFLGMFLYEYARRHPDYSVVLLLRLAKTYETTLEKCCAAADPHECYAKVFDEFKPLVEEPQNLIKQNCELFEQLGEYKFQNALLVRYTKKVPQVSTPTLVEVSRNLGKVGSKCCKHPEAKRMPCAEDYLSVVLNQLCVLHEKTPVSDRVTKCCTESLVNRRPCFSALEVDETYVPKEFNAGTFTFHADICTLSEKERQIKKQTALVELVKHKPKATKEQLKAVMDDFAAFVEKCCKADDKETCFAEEGKKLVAASQAALGL

SEQ ID NO: 138 - protein, 585 aa, Artificial Sequence
  Human Serum Albumin Variant
DAHKSEVAHRFKDLGEENFKALVLIAFAQYLQQCPFEDHVKLVNEVTEFAKTCVADESAENCDKSLHTLFGDKLCTVATLRETYGEMADCCAKQEPERNECFLQHKDDNPNLPRLVRPEVDVMCTAFHDNEETFLKKYLYEIARRHPYFYAPELLFFAKRYKAAFTECCQAADKAACLLPKLDELRDEGKASSAKQRLKCASLQKFGERAFKAWAVARLSQRFPKAEFAEVSKLVTDLTKVHTECCHGDLLECADDRADLAKYICENQDSISSKLKECCEKPLLEKSHCIAEVENDEMPADLPSLAADFVESKDVCKNYAEAKDVFLGMFLYEYARRHPDYSVVLLLRLAKTYETTLEKCCAAADPHECYAKVFDEFKPLVEEPQNLIKQNCELFEQLGEYKFQNALLVRYTKKVPQVSTPTLVEVSRNLGKVGSKCCKHPEAKRMPCAEDYLSVVLNQLCVLHEKTPVSDRVTKCCTESLVNRRPCFSALEVDETYVPKEFNAETFTFHADICTLSEKERQIKKQTALVELVKHKPKATKEQLKAAMDDFAAFVEKCCKADDKETCFAEEGKKLVAASQAALGL

SEQ ID NO: 139 - protein, 585 aa, Artificial Sequence
  Human Serum Albumin Variant
DAHKSEVAHRFKDLGEENFKALVLIAFAQYLQQCPFEDHVKLVNEVTEFAKTCVADESAENCDKSLHTLFGDKLCTVATLRETYGEMADCCAKQEPERNECFLQHKDDNPNLPRLVRPEVDVMCTAFHDNEETFLKKYLYEIARRHPYFYAPELLFFAKRYKAAFTECCQAADKAACLLPKLDELRDEGKASSAKQRLKCASLQKFGERAFKAWAVARLSQRFPKAEFAEVSKLVTDLTKVHTECCHGDLLECADDRADLAKYICENQDSISSKLKECCEKPLLEKSHCIAEVENDEMPADLPSLAADFVESKDVCKNYAEAKDVFLGMFLYEYARRHPDYSVVLLLRLAKTYETTLEKCCAAADPHECYAKVFDEFKPLVEEPQNLIKQNCELFEQLGEYKFQNALLVRYTKKVPQVSTPTLVEVSRNLGKVGSKCCKHPEAKRMPCAEDYLSVVLNQLCVLHEKTPVSDRVTKCCTESLVNRRPCFSALEVDETYVPKEFNAETFTFHADICTLSEKERQIKKQTALVELVKHKPKATKEQLKAVMDDFAAFVEKCCKADDKETCFAEEGYKLVAASQAALGL

SEQ ID NO: 140 - protein, 585 aa, Artificial Sequence
  Human Serum Albumin Variant
DAHKSEVAHRFKDLGEENFKALVLIAFAQYLQQCPFEDHVKLVNEVTEFAKTCVADESAENCDKSLHTLFGDKLCTVATLRETYGEMADCCAKQEPERNECFLQHKDDNPNLPRLVRPEVDVMCTAFHDNEETFLKKYLYEIARRHPYFYAPELLFFAKRYKAAFTECCQAADKAACLLPKLDELRDEGKASSAKQRLKCASLQKFGERAFKAWAVARLSQRFPKAEFAEVSKLVTDLTKVHTECCHGDLLECADDRADLAKYICENQDSISSKLKECCEKPLLEKSHCIAEVENDEMPADLPSLAADFVESKDVCKNYAEAKDVFLGMFLYEYARRHPDYSVVLLLRLAKTYETTLEKCCAAADPHECYAKVFDEFKPLVEEPQNLIKQNCELFEQLGEYKFQNALLVRYTKKVPQVSTPTLIEVSRNLGKVGSKCCKHPEAKRMPCAEDYLSVVLNQLCVLHEKTPVSDRVTKCCTESLVNRRPCFSALEVDETYVPKEFNAETFTFHADICTLSEKERQIKKQTALVELVKHKPKATKEQLKAVMDDFAAFVEKCCKADDKETCFAEEGKKLVAASQAALGL

SEQ ID NO: 141 - protein, 585 aa, Artificial Sequence
  Human Serum Albumin Variant
DAHKSEVAHRFKDLGEENFKALVLIAFAQYLQQCPFEDHVKLVNEVTEFAKTCVADESAENCDKSLHTLFGDKLCTVATLRETYGEMADCCAKQEPERNECFLQHKDDNPNLPRLVRPEVDVMCTAFHDNEETFLKKYLYEIARRHPYFYAPELLFFAKRYKAAFTECCQAADKAACLLPKLDELRDEGKASSAKQRLKCASLQKFGERAFKAWAVARLSQRFPKAEFAEVSKLVTDLTKVHTECCHGDLLECADDRADLAKYICENQDSISSKLKECCEKPLLEKSHCIAEVENDEMPADLPSLAADFVESKDVCKNYAEAKDVFLGMFLYEYARRHPDYSVVLLLRLAKTYETTLEKCCAAADPHECYAKVFDEFKPLVEEPQNLIKQNCELFEQLGEYKFQNALLVRYTKKVPQVSTPTLVEVSRDLGKVGSKCCKHPEAKRMPCAEDYLSVVLNQLCVLHEKTPVSDRVTKCCTESLVNRRPCFSALEVDETYVPKEFNAETFTFHADICTLSEKERQIKKQTALVELVKHKPKATKEQLKAVMDDFAAFVEKCCKADDKETCFAEEGKKLVAASQAALGL

SEQ ID NO: 142 - protein, 585 aa, Artificial Sequence
  Human Serum Albumin Variant
DAHKSEVAHRFKDLGEENFKALVLIAFAQYLQQCPFEDHVKLVNEVTEFAKTCVADESAENCDKSLHTLFGDKLCTVATLRETYGEMADCCAKQEPERNECFLQHKDDNPNLPRLVRPEVDVMCTAFHDNEETFLKKYLYEIARRHPYFYAPELLFFAKRYKAAFTECCQAADKAACLLPKLDELRDEGKASSAKQRLKCASLQKFGERAFKAWAVARLSQRFPKAEFAEVSKLVTDLTKVHTECCHGDLLECADDRADLAKYICENQDSISSKLKECCEKPLLEKSHCIAEVENDEMPADLPSLAADFVESKDVCKNYAEAKDVFLGMFLYEYARRHPDYSVVLLLRLAKTYETTLEKCCAAADPHECYAKVFDEFKPLVEEPQNLIKQNCELFEQLGEYKFQNALLVRYTKKVPQVSTPTLVEVSRNLGKVGSKCCKHPEAKRMPCVEDYLSVVLNQLCVLHEKTPVSDRVTKCCTESLVNRRPCFSALEVDETYVPKEFNAETFTFHADICTLSEKERQIKKQTALVELVKHKPKATKEQLKAVMDDFAAFVEKCCKADDKETCFAEEGKKLVAASQAALGL

SEQ ID NO: 143 - protein, 585 aa, Artificial Sequence
  Human Serum Albumin Variant
DAHKSEVAHRFKDLGEENFKALVLIAFAQYLQQCPFEDHVKLVNEVTEFAKTCVADESAENCDKSLHTLFGDKLCTVATLRETYGEMADCCAKQEPERNECFLQHKDDNPNLPRLVRPEVDVMCTAFHDNEETFLKKYLYEIARRHPYFYAPELLFFAKRYKAAFTECCQAADKAACLLPKLDELRDEGKASSAKQRLKCASLQKFGERAFKAWAVARLSQRFPKAEFAEVSKLVTDLTKVHTECCHGDLLECADDRADLAKYICENQDSISSKLKECCEKPLLEKSHCIAEVENDEMPADLPSLAADFVESKDVCKNYAEAKDVFLGMFLYEYARRHPDYSVVLLLRLAKTYETTLEKCCAAADPHECYAKVFDEFKPLVEEPQNLIKQNCELFEQLGEYKFQNALLVRYTKKVPQVSTPTLVEVSRNLGKVGSKCCKHPEAKRMPCAEDYLSVVLNQLCVLHEKMPVSDRVTKCCTESLVNRRPCFSALEVDETYVPKEFNAETFTFHADICTLSEKERQIKKQTALVELVKHKPKATKEQLKAVMDDFAAFVEKCCKADDKETCFAEEGKKLVAASQAALGL

SEQ ID NO: 144 - protein, 585 aa, Artificial Sequence
  Human Serum Albumin Variant
DAHKSEVAHRFKDLGEENFKALVLIAFAQYLQQCPFEDHVKLVNEVTEFAKTCVADESAENCDKSLHTLFGDKLCTVATLRETYGEMADCCAKQEPERNECFLQHKDDNPNLPRLVRPEVDVMCTAFHDNEETFLKKYLYEIARRHPYFYAPELLFFAKRYKAAFTECCQAADKAACLLPKLDELRDEGKASSAKQRLKCASLQKFGERAFKAWAVARLSQRFPKAEFAEVSKLVTDLTKVHTECCHGDLLECADDRADLAKYICENQDSISSKLKECCEKPLLEKSHCIAEVENDEMPADLPSLAADFVESKDVCKNYAEAKDVFLGMFLYEYARRHPDYSVVLLLRLAKTYETTLEKCCAAADPHECYAKVFDEFKPLVEEPQNLIKQNCELFEQLGEYKFQNALLVRYTKKVPQVSTPTLVEVSRNLGKVGSKCCKHPEAKRMPCAEDYLSVVLNQLCVLHEKTPVSDRVTKCCTESLVNRRPCFSALEVDETYVPKEFNAETFTFHADICTLSEKERQIKKQTALVELVKHKPKATKEQLKAVMDDFTAFVEKCCKADDKETCFAEEGKKLVAASQAALGL

SEQ ID NO: 145 - DNA, 20 bp, Artificial Sequence
  pTAC linearize-F
caagcttggctgttttggcg

SEQ ID NO: 146 - DNA, 25 bp, Artificial Sequence
  pTAC linearize-R
ctatatctccttcttaaagttaaac

SEQ ID NO: 147 - DNA, 34 bp, Artificial Sequence
  tacP-RBS-MCS-rrnBt1t2-F
aagaaggagatatagatgtctgctgtgaaggccg

SEQ ID NO: 148 - DNA, 36 bp, Artificial Sequence
  tacP-RBS-MCS-rrnBt1t2-R
aaacagccaagcttgttacagcttgctcttcagaga

SEQ ID NO: 149 - DNA, 20 bp, Artificial Sequence
  pTAC-sequencing-F
gcctagagcaagacgtttcc

SEQ ID NO: 150 - DNA, 19 bp, Artificial Sequence
  pTAC-sequencing-R
ttaatgcagctggcacgac

SEQ ID NO: 151 - DNA, 23 bp, Artificial Sequence
  Ribosome binding site sequence
tttgtttaactttaagaaggaga

SEQ ID NO: 152 - DNA, 909 bp, Artificial Sequence
  Asp.Uox Variant Coding DNA
atgtctgctgtgaaggccgcaagatatggcaaggataatgtgagggtgtacaaggtgcataaggacgaaaagactggcgtgcagacagtgtacgagatgaccgtgtgcgtcctgctggagggcgaaatcgagacttcttataccaaagccgacaactccgtgattgtggccacagattctatcaagaacactatctatatcaccgccaaacagaacccagtgacaccacctgaactgttcggcagcattctcggcacacactttattgagaagtacaaccacatccatgctgcacacgtgaatatcgtgtgtcatcgctggacccgcatggacatctagggaaagccacacccccactcttttatcagagactctgaagaaaagagaaacgtgcaggtcgacgtggtggagggaaaaggtatcgacatcaagagctcactctccggcctgaccgtgctgaagagtaccaattcacagttttgggggtttctgagagacgaatacactacactgaaggagacttgggatagaatcctgagtaccgacgtggatgcaacctggcagtggaagaatttttccgggctgcaggaagtgcggtcccacgtgcccaagtttgatgcaacctgggcaaccgcaagggaggtgacactgaaaacctttgccgaggacaactccgctagcgtgcaggccacaatgtacaagatggccgaacagatcctggccagacagcagctgattgagactgtggagtactctctgcctaacaagcactatttcgaaatcgacctgtcctggcacaagggactgcagaatactggtaaaaacgcagaggtgttcgcccctcagagtgatcccaatggtctgatcaaatgcacagtggggagatcctctctgaagagcaagctgtaa

SEQ ID NO: 153 - DNA, 909 bp, Artificial Sequence
  Asp.Uox Variant Coding DNA
atgtctgctgtgaaggccgcaagatatggcaaggataatgtgagggtgtacaaggtgcataaggacgaaaagactggcgtgcagacagtgtacgagatgaccgtgtgcgtcctgctggagggcgaaatcgagacttcttataccaaagccgacaactccgtgattgtggccacagattctatcaagaacactatctatatcaccgccaaacagaacccagtgacaccacctgaactgttcggcagcattctcggcacacactttattgagaagtacaaccacatccatgctgcacacgtgaatatcgtgtgtcatcgctggacccgcatggacatcgacggaaagccacacccccactcttttatcagagactctgaagaaaagagaaacgtgcaggtcgacgtggtggagggaaaaggtatcgacatcaagagctcactctccggcctgaccgtgctgaagagtaccaattcacagttttaggggtttctgagagacgaatacactacactgaaggagacttgggatagaatcctgagtaccgacgtggatgcaacctggcagtggaagaatttttccgggctgcaggaagtgcggtcccacgtgcccaagtttgatgcaacctgggcaaccgcaagggaggtgacactgaaaacctttgccgaggacaactccgctagcgtgcaggccacaatgtacaagatggccgaacagatcctggccagacagcagctgattgagactgtggagtactctctgcctaacaagcactatttcgaaatcgacctgtcctggcacaagggactgcagaatactggtaaaaacgcagaggtgttcgcccctcagagtgatcccaatggtctgatcaaatgcacagtggggagatcctctctgaagagcaagctgtaa

SEQ ID NO: 154 - DNA, 909 bp, Artificial Sequence
  Asp.Uox Variant Coding DNA
atgtctgctgtgaaggccgcaagatatggcaaggataatgtgagggtgtacaaggtgcataaggacgaaaagactggcgtgcagacagtgtacgagatgaccgtgtgcgtcctgctggagggcgaaatcgagacttcttataccaaagccgacaactccgtgattgtggccacagattctatcaagaacactatctatatcaccgccaaacagaacccagtgacaccacctgaactgttcggcagcattctcggcacacactttattgagaagtacaaccacatccatgctgcacacgtgaatatcgtgtgtcatcgctggacccgcatggacatcgacggaaagccacacccccactcttttatcagagactctgaagaaaagagaaacgtgcaggtcgacgtggtggagggaaaaggtatcgacatcaagagctcactctccggcctgaccgtgctgaagagtaccaattcacagttttgggggtttctgagagacgaatacactacactgaaggagacttaggatagaatcctgagtaccgacgtggatgcaacctggcagtggaagaatttttccgggctgcaggaagtgcggtcccacgtgcccaagtttgatgcaacctgggcaaccgcaagggaggtgacactgaaaacctttgccgaggacaactccgctagcgtgcaggccacaatgtacaagatggccgaacagatcctggccagacagcagctgattgagactgtggagtactctctgcctaacaagcactatttcgaaatcgacctgtcctggcacaagggactgcagaatactggtaaaaacgcagaggtgttcgcccctcagagtgatcccaatggtctgatcaaatgcacagtggggagatcctctctgaagagcaagctgtaa

SEQ ID NO: 155 - DNA, 912 bp, Artificial Sequence
  Candida.Uox Variant Coding DNA
atgagcaccacactgagcagcagcacctatggtaaagataatgtgaaattcctgaaagtgaaaaaagatccgcagaacccgaaaaaacaagaagttatggaagcaaccgttacctgtctgctggaaggtggttttgataccagctataccgaagcagataatagcagcattgttccgaccgataccgtgaaaaataccattctggttctggcaaaaaccaccgaaatttggccgattgaacgttttgcagccaaactggcaacccattttgttgagaaatattctcatgttagcggtgtgagcgttaaaattgttcaggatcgttgggttaaatatgccgttgatggtaaaccgcatgatcacagctttattcatgaaggtggtgaaaaacgtatcaccgacctgtattacaaacgtagcggtgattataaactgtccagcgcaattaaagatctgaccgttctgaaaagcaccggcagcatgttttagggttataacaaatgcgatttcacaaccctgcagccgaccaccgatcgtattctgagcaccgatgttgatgcaacctgggtttgggataataagaaaattggtagcgtgtacgatattgccaaagcagcagataaaggcatcttcgataatgtgtataatcaggcacgtgaaattaccctgaccacctttgcactggaaaatagcccgagcgttcaggcaaccatgtttaatatggcgacccagattctggaaaaagcgtgtagcgtttatagcgttagctatgcactgccgaacaaacactattttctgattgacctgaaatggaagggccttgaaaatgataacgaactgttttatccgagtccgcatccgaatggtctgattaaatgtaccgttgtgcgtaaagagaaaaccaaactgtaa

SEQ ID NO: 156 - DNA, 912 bp, Artificial Sequence
  Candida.Uox Variant Coding DNA
atgagcaccacactgagcagcagcacctatggtaaagataatgtgaaattcctgaaagtgaaaaaagatccgcagaacccgaaaaaacaagaagttatggaagcaaccgttacctgtctgctggaaggtggttttgataccagctataccgaagcagataatagcagcattgttccgaccgataccgtgaaaaataccattctggttctggcaaaaaccaccgaaatttggccgattgaacgttttgcagccaaactggcaacccattttgttgagaaatattctcatgttagcggtgtgagcgttaaaattgttcaggatcgttgggttaaatatgccgttgatggtaaaccgcatgatcacagctttattcatgaaggtggtgaaaaacgtatcaccgacctgtattacaaacgtagcggtgattataaactgtccagcgcaattaaagatctgaccgttctgaaaagcaccggcagcatgttttatggttataacaaatgcgatttcacaaccctgcagccgaccaccgatcgtattctgagcaccgatgttgatgcaacctgggtttgggataataagaaaattggtagcgtgtaggatattgccaaagcagcagataaaggcatcttcgataatgtgtataatcaggcacgtgaaattaccctgaccacctttgcactggaaaatagcccgagcgttcaggcaaccatgtttaatatggcgacccagattctggaaaaagcgtgtagcgtttatagcgttagctatgcactgccgaacaaacactattttctgattgacctgaaatggaagggccttgaaaatgataacgaactgttttatccgagtccgcatccgaatggtctgattaaatgtaccgttgtgcgtaaagagaaaaccaaactgtaa

SEQ ID NO: 157 - DNA, 912 bp, Artificial Sequence
  Candida.Uox Variant Coding DNA
atgagcaccacactgagcagcagcacctatggtaaagataatgtgaaattcctgaaagtgaaaaaagatccgcagaacccgaaaaaacaagaagttatggaagcaaccgttacctgtctgctggaaggtggttttgataccagctataccgaagcagataatagcagcattgttccgaccgataccgtgaaaaataccattctggttctggcaaaaaccaccgaaatttggccgattgaacgttttgcagccaaactggcaacccattttgttgagaaatattctcatgttagcggtgtgagcgttaaaattgttcaggatcgttgggttaaatatgccgttgatggtaaaccgcatgatcacagctttattcatgaaggtggtgaaaaacgtatcaccgacctgtattacaaacgtagcggtgattataaactgtccagcgcaattaaagatctgaccgttctgaaaagcaccggcagcatgttttatggttataacaaatgcgatttcacaaccctgcagccgaccaccgatcgtattctgagcaccgatgttgatgcaacctgggtttgggataataagaaaattggtagcgtgtacgatattgccaaagcagcagataaaggcatcttcgataatgtgtataatcaggcacgtgaaattaccctgaccacctttgcactggaaaatagcccgagcgttcaggcaaccatgtttaatatggcgacccagattctggaaaaagcgtgtagcgtttatagcgttagctatgcactgccgaacaaacactattttctgattgacctgaaatagaagggccttgaaaatgataacgaactgttttatccgagtccgcatccgaatggtctgattaaatgtaccgttgtgcgtaaagagaaaaccaaactgtaa

SEQ ID NO: 158 - DNA, 909 bp, Artificial Sequence
  Arth.Uox Variant Coding DNA
atgaccgcaaccgcagaaaccagcaccggcaccaaagttgttctgggtcagaatcagtatggtaaagcagaagttcgtctggttaaagttacccgtaataccgcacgtcatgaaattcaggatctgaatgttaccagccagctgcgtggtgattttgaagcagcacataccgcaggcgataatgcacatgttgttgcaaccgatacacagaaaaacaccgtttatgcatttgcccgtgatggttttgcaaccaccgaagaatttctgctgcgtctgggtaaacatttcaccgaaggttttgattgggttaccggtggtcgttgggcagcacagcagtttttctgggatcgtatttaggatcacgatcatgcctttagccgcaataaaagcgaagtgcgtaccgcagttctggaaattagcggtagcgaacaggcaattgttgcaggtattgaaggtctgaccgttctgaaaagcaccggtagcgagtttcatggttttccgcgtgataaatacaccacactgcaagaaaccaccgatcgtattctggcaaccgatgttagcgcacgttggcgttataataccgttgaagttgattttgatgcggtttatgcaagcgttcgtggtctgctgctgaaagcatttgcagaaacccatagcctggcactgcagcagacaatgtatgaaatgggtcgtgcagttattgaaacccatccggaaattgatgagatcaaaatgagcctgccgaacaaacatcattttctggttgatctgcagccgtttggtcaggataatccgaatgaagtgttttatgcagcagatcgtccgtatggtctgattgaagcaaccattcagcgtgaaggtagccgtgcagatcatccgatttggagtaatattgcaggtttttgctaa

SEQ ID NO: 159 - DNA, 909 bp, Artificial Sequence
  Arth.Uox Variant Coding DNA
atgaccgcaaccgcagaaaccagcaccggcaccaaagttgttctgggtcagaatcagtatggtaaagcagaagttcgtctggttaaagttacccgtaataccgcacgtcatgaaattcaggatctgaatgttaccagccagctgcgtggtgattttgaagcagcacataccgcaggcgataatgcacatgttgttgcaaccgatacacagaaaaacaccgtttatgcatttgcccgtgatggttttgcaaccaccgaagaatttctgctgcgtctgggtaaacatttcaccgaaggttttgattgggttaccggtggtcgttgggcagcacagcagtttttctgggatcgtattaatgatcacgatcatgcctttagccgcaataaaagcgaagtgcgtaccgcagttctggaaattagcggttaggaacaggcaattgttgcaggtattgaaggtctgaccgttctgaaaagcaccggtagcgagtttcatggttttccgcgtgataaatacaccacactgcaagaaaccaccgatcgtattctggcaaccgatgttagcgcacgttggcgttataataccgttgaagttgattttgatgcggtttatgcaagcgttcgtggtctgctgctgaaagcatttgcagaaacccatagcctggcactgcagcagacaatgtatgaaatgggtcgtgcagttattgaaacccatccggaaattgatgagatcaaaatgagcctgccgaacaaacatcattttctggttgatctgcagccgtttggtcaggataatccgaatgaagtgttttatgcagcagatcgtccgtatggtctgattgaagcaaccattcagcgtgaaggtagccgtgcagatcatccgatttggagtaatattgcaggtttttgctaa

SEQ ID NO: 160 - DNA, 909 bp, Artificial Sequence
  Arth.Uox Variant Coding DNA
atgaccgcaaccgcagaaaccagcaccggcaccaaagttgttctgggtcagaatcagtatggtaaagcagaagttcgtctggttaaagttacccgtaataccgcacgtcatgaaattcaggatctgaatgttaccagccagctgcgtggtgattttgaagcagcacataccgcaggcgataatgcacatgttgttgcaaccgatacacagaaaaacaccgtttatgcatttgcccgtgatggttttgcaaccaccgaagaatttctgctgcgtctgggtaaacatttcaccgaaggttttgattgggttaccggtggtcgttgggcagcacagcagtttttctgggatcgtattaatgatcacgatcatgcctttagccgcaataaaagcgaagtgcgtaccgcagttctggaaattagcggtagcgaacaggcaattgttgcaggtattgaaggtctgaccgttctgaaaagcaccggtagcgagtttcatggttttccgcgtgataaatacaccacactgcaagaaaccaccgatcgtattctggcaaccgatgttagcgcacgttggcgttataataccgtttaggttgattttgatgcggtttatgcaagcgttcgtggtctgctgctgaaagcatttgcagaaacccatagcctggcactgcagcagacaatgtatgaaatgggtcgtgcagttattgaaacccatccggaaattgatgagatcaaaatgagcctgccgaacaaacatcattttctggttgatctgcagccgtttggtcaggataatccgaatgaagtgttttatgcagcagatcgtccgtatggtctgattgaagcaaccattcagcgtgaaggtagccgtgcagatcatccgatttggagtaatattgcaggtttttgctaa

SEQ ID NO: 161 - DNA, 25 bp, Artificial Sequence
  pBAD-AgUox_F
gccgccatggtgtctgctgtgaagg

SEQ ID NO: 162 - DNA, 25 bp, Artificial Sequence
  pBAD-AgUox_R
gccgagatctttaatggtgatggtg

SEQ ID NO: 163 - DNA, 37 bp, Artificial Sequence
  AgUox-196Amb_F
gtcgaagtccacctatacggtgttgtaacgccaacgg

SEQ ID NO: 164 - DNA, 37 bp, Artificial Sequence
  AgUox-196Amb_R
ccgttggcgttacaacaccgtataggtggacttcgac

SEQ ID NO: 165 - protein, 16 aa, Artificial Sequence
  AgUox-WT fregment
YNTVEVDFDAVYASVR

SEQ ID NO: 166 - protein, 16 aa, Artificial Sequence
  AgUox-frTet fregment
YNTVXVDFDAVYASVR

SEQ ID NO: 167 - protein, 19 aa, Artificial Sequence
  fregment control
AVIETHPEIDEIKMSLPNK